European Patent Specification EP 3 538 559 B1, published April 9, 2025. Title: RECOMBINANT PMHC CLASS II MOLECULES. Applicant: UTI LIMITED PARTNERSHIP. The sequence listing filed with the application follows.

SEQUENCE LISTING (65 sequences)

SEQ ID NO: 1 - DNA, 3171 bp, Artificial Sequence
  source: /note="Description of Artificial Sequence: Synthetic polynucleotide"
atgggttctctgcaaccgctggccaccttgtacctgctgggtatgctggtcgctagcagcctcggacagcacctgcagaaggactacagagcctactacaccttcggaggtggaggcggctcaggaggtggaagcggcggctctggggacacccgaccacgtttcttggagtactctacgtctgagtgtcatttcttcaatgggacggagcgggtgcggtacctggacagatacttccataaccaggaggagaacgtgcgcttcgacagcgacgtgggggagttccgggcggtgacggagctggggcggcctgatgccgagtactggaacagccagaaggacctcctggagcagaagcggggccgggtggacaactactgcagacacaactacggggttgtggagagcttcacagtgcagcggcgagtccatcctaaggtgactgtgtatccttcaaagacccagcccctgcagcaccataacctcctggtctgttctgtgagtggtttctatccaggcagcattgaagtcaggtggttccggaatggccaggaagagaagactggggtggtgtccacaggcctgatccacaatggagactggaccttccagaccctggtgatgctggaaacagttcctcggagtggagaggtttacacctgccaagtggagcacccaagcgtgacaagccctctcacagtggaatggagagcacggtctgaatctgcacagagcaagtccggaggcggaggcggacggatcgctcggctagaggaaaaagtgaaaaccttgaaagcgcaaaactccgagctggcgtccacggccaacatgctcagggaacaggtggcacagcttaagcagaaagtcatgaaccacgacaaaactcacacatgcccaccgtgcccagcacctgaactcctggggggaccgtcagtcttcctcttccccccaaaacccaaggacaccctcatgatctcccggacccctgaggtcacatgcgtggtggtggacgtgagccacgaagaccctgaggtcaagttcaactggtacgtggacggcgtggaggtgcataatgccaagacaaagccgcgggaggagcagtacaacagcacgtaccgtgtggtcagcgtcctcaccgtcctgcaccaggactggctgaatggcaaggagtacaagtgcaaagtctccaacaaagccctcccagcccccatcgagaaaaccatctccaaagccaaagggcagccccgagaaccacaggtgtgcaccctgcccccatcccgggatgagctgaccaagaaccaggtcagcctgagctgcgcggtcaaaggcttctatcccagcgacatcgccgtggagtgggagagcaatgggcagccggagaacaactacaagaccacgcctcccgtgctggactccgacggctccttcttcctcgtcagcaagctcaccgtggacaagagcaggtggcagcaggggaacgtcttctcatgctccgtgatgcatgaggctctgcacaaccactacacacagaagagcctctccctgtctcccggcggctccggagccacgaacttctctctgttaaagcaagcaggagacgtggaagaaaaccccggtcccatggctatcatctacctcatcctcctgttcaccgctgtgcggggcatcaaagaagaacatgtgatcatccaggccgagttctatctgaatcctgaccaatcaggcgagtttatgtttgactttgatggtgatgagattttccatgtggatatggcaaagaaggagacggtctggcggcttgaagaatttggacgatttgccagctttgaggctcaaggtgcattggccaacatagctgtggacaaagccaacctggaaatcatgacaaagcgctccaactatactccgatcaccaatgtacctccagaggtaactgtgctcacaaacagccctgtggaactgagagagcccaacgtcctcatctgtttcatagacaagttcaccccaccagtggtcaatgtcacgtggcttcgaaatggaaaacctgtcaccacaggagtgtcagagacagtcttcctgcccagggaagaccaccttttccgcaagttccactatctccccttcctgccctcaactgaggacgtttacgactgcagggtggagcactggggcttggatgagcctcttctcaagcactgggagtttgatgctccaagccctctcccagagactacagagtccggaggcggaggcggactgacagatacactccaagcggagacagatcaacttgaagacgagaagtctgcgttgcagaccgagattgccaatctactgaaagagaaggaaaaactggagtttattttggcagcccacgacaaaactcacacatgcccaccgtgcccagcacctgaactcctggggggaccgtcagtcttcctcttccccccaaaacccaaggacaccctcatgatctcccggacccctgaggtcacatgcgtggtggtggacgtgagccacgaagaccctgaggtcaagttcaactggtacgtggacggcgtggaggtgcataatgccaagacaaagccgcgggaggagcagtacaacagcacgtaccgtgtggtcagcgtcctcaccgtcctgcaccaggactggctgaatggcaaggagtacaagtgcaaagtctccaacaaagccctcccagcccccatcgagaaaaccatctccaaagccaaagggcagccccgagaaccacaggtgtacaccctgcccccatgccgggatgagctgaccaagaaccaggtcagcctgtggtgcctggtcaaaggcttctatcccagcgacatcgccgtggagtgggagagcaatgggcagccggagaacaactacaagaccacgcctcccgtgctggactccgacggctccttcttcctctacagcaagctcaccgtggacaagagcaggtggcagcaggggaacgtcttctcatgctccgtgatgcatgaggctctgcacaaccactacacacagaagagcctctccctgtctccgggcggtagtggtagtggtagtggatctctgggtggtatcttcgaggctatgaagatggagctgcgcgatcaccatcaccatcaccataactggagccaccctcagttcgagaagtgttga

SEQ ID NO: 2 - DNA, 2931 bp, Artificial Sequence
  source: /note="Description of Artificial Sequence: Synthetic polynucleotide"
atgggttctctgcaaccgctggccaccttgtacctgctgggtatgctggtcgctagcagcctcggacagcacctgcagaaggactacagagcctactacaccttcggaggtggaggcggctcaggaggtggaagcggcggctctggggacacccgaccacgtttcttggagtactctacgtctgagtgtcatttcttcaatgggacggagcgggtgcggtacctggacagatacttccataaccaggaggagaacgtgcgcttcgacagcgacgtgggggagttccgggcggtgacggagctggggcggcctgatgccgagtactggaacagccagaaggacctcctggagcagaagcggggccgggtggacaactactgcagacacaactacggggttgtggagagcttcacagtgcagcggcgagtccatcctaaggtgactgtgtatccttcaaagacccagcccctgcagcaccataacctcctggtctgttctgtgagtggtttctatccaggcagcattgaagtcaggtggttccggaatggccaggaagagaagactggggtggtgtccacaggcctgatccacaatggagactggaccttccagaccctggtgatgctggaaacagttcctcggagtggagaggtttacacctgccaagtggagcacccaagcgtgacaagccctctcacagtggaatggagagcacggtctgaatctgcacagagcaagtccggaggcggaggcggagacaaaactcacacatgcccaccgtgcccagcacctgaactcctggggggaccgtcagtcttcctcttccccccaaaacccaaggacaccctcatgatctcccggacccctgaggtcacatgcgtggtggtggacgtgagccacgaagaccctgaggtcaagttcaactggtacgtggacggcgtggaggtgcataatgccaagacaaagccgcgggaggagcagtacaacagcacgtaccgtgtggtcagcgtcctcaccgtcctgcaccaggactggctgaatggcaaggagtacaagtgcaaagtctccaacaaagccctcccagcccccatcgagaaaaccatctccaaagccaaagggcagccccgagaaccacaggtgtgcaccctgcccccatcccgggatgagctgaccaagaaccaggtcagcctgagctgcgcggtcaaaggcttctatcccagcgacatcgccgtggagtgggagagcaatgggcagccggagaacaactacaagaccacgcctcccgtgctggactccgacggctccttcttcctcgtcagcaagctcaccgtggacaagagcaggtggcagcaggggaacgtcttctcatgctccgtgatgcatgaggctctgcacaaccactacacacagaagagcctctccctgtctcccggcggctccggagccacgaacttctctctgttaaagcaagcaggagacgtggaagaaaaccccggtcccatggctatcatctacctcatcctcctgttcaccgctgtgcggggcatcaaagaagaacatgtgatcatccaggccgagttctatctgaatcctgaccaatcaggcgagtttatgtttgactttgatggtgatgagattttccatgtggatatggcaaagaaggagacggtctggcggcttgaagaatttggacgatttgccagctttgaggctcaaggtgcattggccaacatagctgtggacaaagccaacctggaaatcatgacaaagcgctccaactatactccgatcaccaatgtacctccagaggtaactgtgctcacaaacagccctgtggaactgagagagcccaacgtcctcatctgtttcatagacaagttcaccccaccagtggtcaatgtcacgtggcttcgaaatggaaaacctgtcaccacaggagtgtcagagacagtcttcctgcccagggaagaccaccttttccgcaagttccactatctccccttcctgccctcaactgaggacgtttacgactgcagggtggagcactggggcttggatgagcctcttctcaagcactgggagtttgatgctccaagccctctcccagagactacagagtccggaggcggaggcggagacaaaactcacacatgcccaccgtgcccagcacctgaactcctggggggaccgtcagtcttcctcttccccccaaaacccaaggacaccctcatgatctcccggacccctgaggtcacatgcgtggtggtggacgtgagccacgaagaccctgaggtcaagttcaactggtacgtggacggcgtggaggtgcataatgccaagacaaagccgcgggaggagcagtacaacagcacgtaccgtgtggtcagcgtcctcaccgtcctgcaccaggactggctgaatggcaaggagtacaagtgcaaagtctccaacaaagccctcccagcccccatcgagaaaaccatctccaaagccaaagggcagccccgagaaccacaggtgtacaccctgcccccatgccgggatgagctgaccaagaaccaggtcagcctgtggtgcctggtcaaaggcttctatcccagcgacatcgccgtggagtgggagagcaatgggcagccggagaacaactacaagaccacgcctcccgtgctggactccgacggctccttcttcctctacagcaagctcaccgtggacaagagcaggtggcagcaggggaacgtcttctcatgctccgtgatgcatgaggctctgcacaaccactacacacagaagagcctctccctgtctccgggcggtagtggtagtggtagtggatctctgggtggtatcttcgaggctatgaagatggagctgcgcgatcaccatcaccatcaccataactggagccaccctcagttcgagaagtgttga

SEQ ID NO: 3 - DNA, 3168 bp, Artificial Sequence
  source: /note="Description of Artificial Sequence: Synthetic polynucleotide"
atggctatcatctacctcatcctcctgttcaccgctgtgcggggcagatctgcccaccatcccatctgggcccgaatggacgccggaggtggaggctcactagtgccccgaggctctggaggtggaggctctggagactccgaaaggcatttcgtgcaccagttcaagggcgagtgctacttcaccaacgggacgcagcgcatacggctcgtgaccagatacatctacaaccgggaggagtacctgcgcttcgacagcgacgtgggcgagtaccgcgcggtgaccgagctggggcggcactcagccgagtactacaataagcagtacctggagcgaacgcgggccgagctggacacggcgtgcagacacaactacgaggagacggaggtccccacctccctgcggcggcttgaacagcccaatgtcgccatctccctgtccaggacagaggccctcaaccaccacaacactctggtctgttcggtgacagatttctacccagccaagatcaaagtgcgctggttcaggaatggccaggaggagacagtgggggtctcatccacacagcttattaggaatggggactggaccttccaggtcctggtcatgctggagatgacccctcatcagggagaggtctatacctgccatgtggagcatcccagcctgaagagccccatcactgtggagtggagggcacagtccgagtctgcccggagcaagtccggaggcggaggcggacggatcgctcggctagaggaaaaagtgaaaaccttgaaagcgcaaaactccgagctggcgtccacggccaacatgctcagggaacaggtggcacagcttaagcagaaagtcatgaaccacgacaaaactcacacatgcccaccgtgcccagcacctgaactcctggggggaccgtcagtcttcctcttccccccaaaacccaaggacaccctcatgatctcccggacccctgaggtcacatgcgtggtggtggacgtgagccacgaagaccctgaggtcaagttcaactggtacgtggacggcgtggaggtgcataatgccaagacaaagccgcgggaggagcagtacaacagcacgtaccgtgtggtcagcgtcctcaccgtcctgcaccaggactggctgaatggcaaggagtacaagtgcaaggtctccaacaaagccctcccagcccccatcgagaaaaccatctccaaagccaaagggcagccccgagaaccacaggtgtgcaccctgcccccatcccgggatgagctgaccaagaaccaggtcagcctgagctgcgcggtcaaaggcttctatcccagcgacatcgccgtggagtgggagagcaatgggcagccggagaacaactacaagaccacgcctcccgtgctggactccgacggctccttcttcctcgtcagcaagctcaccgtggacaagagtaggtggcagcaggggaacgtcttctcatgctccgtgatgcatgaggctctgcacaaccactacacacagaagagcctctccctgtctcccggcggctccggagccacgaacttctctctgttaaagcaagcaggagacgtggaagaaaaccccggtcccatggctatcatctacctcatcctcctgttcaccgctgtgcggggcgaagacgacattgaggccgaccacgtaggcttctatggtacaactgtttatcagtctcctggagacattggccagtacacacatgaatttgatggtgatgagttgttctatgtggacttggataagaagaaaactgtctggaggcttcctgagtttggccaattgatactctttgagccccaaggtggactgcaaaacatagctgcagaaaaacacaacttgggaatcttgactaagaggtcaaatttcaccccagctaccaatgaggctcctcaagcgactgtgttccccaagtcccctgtgctgctgggtcagcccaacacccttatctgctttgtggacaacatcttcccacctgtgatcaacatcacatggctcagaaatagcaagtcagtcacagacggcgtttatgagaccagcttcctcgtcaaccgtgaccattccttccacaagctgtcttatctcaccttcatcccttctgatgatgacatttatgactgcaaggtggagcactggggcctggaggagccggttctgaaacactgggaacctgagattccagcccccatgtcagagctgacagagtccggaggcggaggcggactgacagatacactccaagcggagacagatcaacttgaagacgagaagtctgcgttgcagaccgagattgccaatctactgaaagagaaggaaaaactggagtttattttggcagcccacgacaaaactcacacatgcccaccgtgcccagcacctgaactcctggggggaccgtcagtcttcctcttccccccaaaacccaaggacaccctcatgatctcccggacccctgaggtcacatgcgtggtggtggacgtgagccacgaagaccctgaggtcaagttcaactggtacgtggacggcgtggaggtgcataatgccaagacaaagccgcgggaggagcagtacaacagcacgtaccgtgtggtcagcgtcctcaccgtcctgcaccaggactggctgaatggcaaggagtacaagtgcaaggtctccaacaaagccctcccagcccccatcgagaaaaccatctccaaagccaaagggcagccccgagaaccacaggtgtacaccctgcccccatgccgggatgagctgaccaagaaccaggtcagcctgtggtgcctggtcaaaggcttctatcccagcgacatcgccgtggagtgggagagcaatgggcagccggagaacaactacaagaccacgcctcccgtgctggactccgacggctccttcttcctctacagcaagctcaccgtggacaagagtaggtggcagcaggggaacgtcttctcatgctccgtgatgcatgaggctctgcacaaccactacacacagaagagcctctccctgtctccgggcggtagtggtagtggtagtggatctctgggtggtatcttcgaggctatgaagatggagctgcgcgatcaccatcaccatcaccataactggagccaccctcagttcgagaagtgttga

SEQ ID NO: 4 - DNA, 2928 bp, Artificial Sequence
  source: /note="Description of Artificial Sequence: Synthetic polynucleotide"
atggctatcatctacctcatcctcctgttcaccgctgtgcggggcagatctgcccaccatcccatctgggcccgaatggacgccggaggtggaggctcactagtgccccgaggctctggaggtggaggctctggagactccgaaaggcatttcgtgcaccagttcaagggcgagtgctacttcaccaacgggacgcagcgcatacggctcgtgaccagatacatctacaaccgggaggagtacctgcgcttcgacagcgacgtgggcgagtaccgcgcggtgaccgagctggggcggcactcagccgagtactacaataagcagtacctggagcgaacgcgggccgagctggacacggcgtgcagacacaactacgaggagacggaggtccccacctccctgcggcggcttgaacagcccaatgtcgccatctccctgtccaggacagaggccctcaaccaccacaacactctggtctgttcggtgacagatttctacccagccaagatcaaagtgcgctggttcaggaatggccaggaggagacagtgggggtctcatccacacagcttattaggaatggggactggaccttccaggtcctggtcatgctggagatgacccctcatcagggagaggtctatacctgccatgtggagcatcccagcctgaagagccccatcactgtggagtggagggcacagtccgagtctgcccggagcaagtccggaggcggaggcggagacaaaactcacacatgcccaccgtgcccagcacctgaactcctggggggaccgtcagtcttcctcttccccccaaaacccaaggacaccctcatgatctcccggacccctgaggtcacatgcgtggtggtggacgtgagccacgaagaccctgaggtcaagttcaactggtacgtggacggcgtggaggtgcataatgccaagacaaagccgcgggaggagcagtacaacagcacgtaccgtgtggtcagcgtcctcaccgtcctgcaccaggactggctgaatggcaaggagtacaagtgcaaggtctccaacaaagccctcccagcccccatcgagaaaaccatctccaaagccaaagggcagccccgagaaccacaggtgtgcaccctgcccccatcccgggatgagctgaccaagaaccaggtcagcctgagctgcgcggtcaaaggcttctatcccagcgacatcgccgtggagtgggagagcaatgggcagccggagaacaactacaagaccacgcctcccgtgctggactccgacggctccttcttcctcgtcagcaagctcaccgtggacaagagtaggtggcagcaggggaacgtcttctcatgctccgtgatgcatgaggctctgcacaaccactacacacagaagagcctctccctgtctcccggcggctccggagccacgaacttctctctgttaaagcaagcaggagacgtggaagaaaaccccggtcccatggctatcatctacctcatcctcctgttcaccgctgtgcggggcgaagacgacattgaggccgaccacgtaggcttctatggtacaactgtttatcagtctcctggagacattggccagtacacacatgaatttgatggtgatgagttgttctatgtggacttggataagaagaaaactgtctggaggcttcctgagtttggccaattgatactctttgagccccaaggtggactgcaaaacatagctgcagaaaaacacaacttgggaatcttgactaagaggtcaaatttcaccccagctaccaatgaggctcctcaagcgactgtgttccccaagtcccctgtgctgctgggtcagcccaacacccttatctgctttgtggacaacatcttcccacctgtgatcaacatcacatggctcagaaatagcaagtcagtcacagacggcgtttatgagaccagcttcctcgtcaaccgtgaccattccttccacaagctgtcttatctcaccttcatcccttctgatgatgacatttatgactgcaaggtggagcactggggcctggaggagccggttctgaaacactgggaacctgagattccagcccccatgtcagagctgacagagtccggaggcggaggcggagacaaaactcacacatgcccaccgtgcccagcacctgaactcctggggggaccgtcagtcttcctcttccccccaaaacccaaggacaccctcatgatctcccggacccctgaggtcacatgcgtggtggtggacgtgagccacgaagaccctgaggtcaagttcaactggtacgtggacggcgtggaggtgcataatgccaagacaaagccgcgggaggagcagtacaacagcacgtaccgtgtggtcagcgtcctcaccgtcctgcaccaggactggctgaatggcaaggagtacaagtgcaaggtctccaacaaagccctcccagcccccatcgagaaaaccatctccaaagccaaagggcagccccgagaaccacaggtgtacaccctgcccccatgccgggatgagctgaccaagaaccaggtcagcctgtggtgcctggtcaaaggcttctatcccagcgacatcgccgtggagtgggagagcaatgggcagccggagaacaactacaagaccacgcctcccgtgctggactccgacggctccttcttcctctacagcaagctcaccgtggacaagagtaggtggcagcaggggaacgtcttctcatgctccgtgatgcatgaggctctgcacaaccactacacacagaagagcctctccctgtctccgggcggtagtggtagtggtagtggatctctgggtggtatcttcgaggctatgaagatggagctgcgcgatcaccatcaccatcaccataactggagccaccctcagttcgagaagtgttga

SEQ ID NO: 5 - DNA, 3168 bp, Artificial Sequence
  source: /note="Description of Artificial Sequence: Synthetic polynucleotide"
atgggttctctgcaaccgctggccaccttgtacctgctgggtatgctggtcgctagcagcctcggacagcacctgcagaaggactacagagcctactacaccttcggaggtggaggcggctcaggaggtggaagcggcggctctggggacacccgaccacgtttcttggagtactctacgtctgagtgtcatttcttcaatgggacggagcgggtgcggtacctggacagatacttccataaccaggaggagaacgtgcgcttcgacagcgacgtgggggagttccgggcggtgacggagctggggcggcctgatgccgagtactggaacagccagaaggacctcctggagcagaagcggggccgggtggacaactactgcagacacaactacggggttgtggagagcttcacagtgcagcggcgagtccatcctaaggtgactgtgtatccttcaaagacccagcccctgcagcaccataacctcctggtctgttctgtgagtggtttctatccaggcagcattgaagtcaggtggttccggaatggccaggaagagaagactggggtggtgtccacaggcctgatccacaatggagactggaccttccagaccctggtgatgctggaaacagttcctcggagtggagaggtttacacctgccaagtggagcacccaagcgtgacaagccctctcacagtggaatggagagcacggtctgaatctgcacagagcaagtccggaggcggaggcggacggatcgctcggctagaggaaaaagtgaaaaccttgaaagcgcaaaactccgagctggcgtccacggccaacatgctcagggaacaggtggcacagcttaagcagaaagtcatgaaccacgacaaaactcacacatgcccaccgtgcccagcacctgaactcctggggggaccgtcagtcttcctcttccccccaaaacccaaggacaccctcatgatctcccggacccctgaggtcacatgcgtggtggtggacgtgagccacgaagaccctgaggtcaagttcaactggtacgtggacggcgtggaggtgcataatgccaagacaaagccgcgggaggagcagtacaacagcacgtaccgtgtggtcagcgtcctcaccgtcctgcaccaggactggctgaatggcaaggagtacaagtgcaaagtctccaacaaagccctcccagcccccatcgagaaaaccatctccaaagccaaagggcagccccgagaaccacaggtgtacaccctgcccccatgccgggatgagctgaccaagaaccaggtcagcctgtggtgcctggtcaaaggcttctatcccagcgacatcgccgtggagtgggagagcaatgggcagccggagaacaactacaagaccacgcctcccgtgctggactccgacggctccttcttcctctacagcaagctcaccgtggacaagagcaggtggcagcaggggaacgtcttctcatgctccgtgatgcatgaggctctgcacaaccactacacacagaagagcctctccctgtctccgggcggctccggagccacgaacttctctctgttaaagcaagcaggagacgtggaagaaaaccccggtcccatggctatcatctacctcatcctcctgttcaccgctgtgcggggcatcaaagaagaacatgtgatcatccaggccgagttctatctgaatcctgaccaatcaggcgagtttatgtttgactttgatggtgatgagattttccatgtggatatggcaaagaaggagacggtctggcggcttgaagaatttggacgatttgccagctttgaggctcaaggtgcattggccaacatagctgtggacaaagccaacctggaaatcatgacaaagcgctccaactatactccgatcaccaatgtacctccagaggtaactgtgctcacaaacagccctgtggaactgagagagcccaacgtcctcatctgtttcatagacaagttcaccccaccagtggtcaatgtcacgtggcttcgaaatggaaaacctgtcaccacaggagtgtcagagacagtcttcctgcccagggaagaccaccttttccgcaagttccactatctccccttcctgccctcaactgaggacgtttacgactgcagggtggagcactggggcttggatgagcctcttctcaagcactgggagtttgatgctccaagccctctcccagagactacagagtccggaggcggaggcggactgacagatacactccaagcggagacagatcaacttgaagacgagaagtctgcgttgcagaccgagattgccaatctactgaaagagaaggaaaaactggagtttattttggcagcccacgacaaaactcacacatgcccaccgtgcccagcacctgaactcctggggggaccgtcagtcttcctcttccccccaaaacccaaggacaccctcatgatctcccggacccctgaggtcacatgcgtggtggtggacgtgagccacgaagaccctgaggtcaagttcaactggtacgtggacggcgtggaggtgcataatgccaagacaaagccgcgggaggagcagtacaacagcacgtaccgtgtggtcagcgtcctcaccgtcctgcaccaggactggctgaatggcaaggagtacaagtgcaaagtctccaacaaagccctcccagcccccatcgagaaaaccatctccaaagccaaagggcagccccgagaaccacaggtgtgcaccctgcccccatcccgggatgagctgaccaagaaccaggtcagcctgagctgcgcggtcaaaggcttctatcccagcgacatcgccgtggagtgggagagcaatgggcagccggagaacaactacaagaccacgcctcccgtgctggactccgacggctccttcttcctcgtcagcaagctcaccgtggacaagagcaggtggcagcaggggaacgtcttctcatgctccgtgatgcatgaggctctgcacaaccactacacacagaagagcctctccctgtctcccggcggtagtggtagtggtagtggatctctgggtggtatcttcgaggctatgaagatggagctgcgcgatcaccatcaccatcaccataactggagccaccctcagttcgagaagtgt

SEQ ID NO: 6 - DNA, 2928 bp, Artificial Sequence
  source: /note="Description of Artificial Sequence: Synthetic polynucleotide"
atgggttctctgcaaccgctggccaccttgtacctgctgggtatgctggtcgctagcagcctcggacagcacctgcagaaggactacagagcctactacaccttcggaggtggaggcggctcaggaggtggaagcggcggctctggggacacccgaccacgtttcttggagtactctacgtctgagtgtcatttcttcaatgggacggagcgggtgcggtacctggacagatacttccataaccaggaggagaacgtgcgcttcgacagcgacgtgggggagttccgggcggtgacggagctggggcggcctgatgccgagtactggaacagccagaaggacctcctggagcagaagcggggccgggtggacaactactgcagacacaactacggggttgtggagagcttcacagtgcagcggcgagtccatcctaaggtgactgtgtatccttcaaagacccagcccctgcagcaccataacctcctggtctgttctgtgagtggtttctatccaggcagcattgaagtcaggtggttccggaatggccaggaagagaagactggggtggtgtccacaggcctgatccacaatggagactggaccttccagaccctggtgatgctggaaacagttcctcggagtggagaggtttacacctgccaagtggagcacccaagcgtgacaagccctctcacagtggaatggagagcacggtctgaatctgcacagagcaagtccggaggcggaggcggagacaaaactcacacatgcccaccgtgcccagcacctgaactcctggggggaccgtcagtcttcctcttccccccaaaacccaaggacaccctcatgatctcccggacccctgaggtcacatgcgtggtggtggacgtgagccacgaagaccctgaggtcaagttcaactggtacgtggacggcgtggaggtgcataatgccaagacaaagccgcgggaggagcagtacaacagcacgtaccgtgtggtcagcgtcctcaccgtcctgcaccaggactggctgaatggcaaggagtacaagtgcaaagtctccaacaaagccctcccagcccccatcgagaaaaccatctccaaagccaaagggcagccccgagaaccacaggtgtacaccctgcccccatgccgggatgagctgaccaagaaccaggtcagcctgtggtgcctggtcaaaggcttctatcccagcgacatcgccgtggagtgggagagcaatgggcagccggagaacaactacaagaccacgcctcccgtgctggactccgacggctccttcttcctctacagcaagctcaccgtggacaagagcaggtggcagcaggggaacgtcttctcatgctccgtgatgcatgaggctctgcacaaccactacacacagaagagcctctccctgtctccgggcggctccggagccacgaacttctctctgttaaagcaagcaggagacgtggaagaaaaccccggtcccatggctatcatctacctcatcctcctgttcaccgctgtgcggggcatcaaagaagaacatgtgatcatccaggccgagttctatctgaatcctgaccaatcaggcgagtttatgtttgactttgatggtgatgagattttccatgtggatatggcaaagaaggagacggtctggcggcttgaagaatttggacgatttgccagctttgaggctcaaggtgcattggccaacatagctgtggacaaagccaacctggaaatcatgacaaagcgctccaactatactccgatcaccaatgtacctccagaggtaactgtgctcacaaacagccctgtggaactgagagagcccaacgtcctcatctgtttcatagacaagttcaccccaccagtggtcaatgtcacgtggcttcgaaatggaaaacctgtcaccacaggagtgtcagagacagtcttcctgcccagggaagaccaccttttccgcaagttccactatctccccttcctgccctcaactgaggacgtttacgactgcagggtggagcactggggcttggatgagcctcttctcaagcactgggagtttgatgctccaagccctctcccagagactacagagtccggaggcggaggcggagacaaaactcacacatgcccaccgtgcccagcacctgaactcctggggggaccgtcagtcttcctcttccccccaaaacccaaggacaccctcatgatctcccggacccctgaggtcacatgcgtggtggtggacgtgagccacgaagaccctgaggtcaagttcaactggtacgtggacggcgtggaggtgcataatgccaagacaaagccgcgggaggagcagtacaacagcacgtaccgtgtggtcagcgtcctcaccgtcctgcaccaggactggctgaatggcaaggagtacaagtgcaaagtctccaacaaagccctcccagcccccatcgagaaaaccatctccaaagccaaagggcagccccgagaaccacaggtgtgcaccctgcccccatcccgggatgagctgaccaagaaccaggtcagcctgagctgcgcggtcaaaggcttctatcccagcgacatcgccgtggagtgggagagcaatgggcagccggagaacaactacaagaccacgcctcccgtgctggactccgacggctccttcttcctcgtcagcaagctcaccgtggacaagagcaggtggcagcaggggaacgtcttctcatgctccgtgatgcatgaggctctgcacaaccactacacacagaagagcctctccctgtctcccggcggtagtggtagtggtagtggatctctgggtggtatcttcgaggctatgaagatggagctgcgcgatcaccatcaccatcaccataactggagccaccctcagttcgagaagtgt

SEQ ID NO: 7 - DNA, 3165 bp, Artificial Sequence
  source: /note="Description of Artificial Sequence: Synthetic polynucleotide"
atggctatcatctacctcatcctcctgttcaccgctgtgcggggcagatctgcccaccatcccatctgggcccgaatggacgccggaggtggaggctcactagtgccccgaggctctggaggtggaggctctggagactccgaaaggcatttcgtgcaccagttcaagggcgagtgctacttcaccaacgggacgcagcgcatacggctcgtgaccagatacatctacaaccgggaggagtacctgcgcttcgacagcgacgtgggcgagtaccgcgcggtgaccgagctggggcggcactcagccgagtactacaataagcagtacctggagcgaacgcgggccgagctggacacggcgtgcagacacaactacgaggagacggaggtccccacctccctgcggcggcttgaacagcccaatgtcgccatctccctgtccaggacagaggccctcaaccaccacaacactctggtctgttcggtgacagatttctacccagccaagatcaaagtgcgctggttcaggaatggccaggaggagacagtgggggtctcatccacacagcttattaggaatggggactggaccttccaggtcctggtcatgctggagatgacccctcatcagggagaggtctatacctgccatgtggagcatcccagcctgaagagccccatcactgtggagtggagggcacagtccgagtctgcccggagcaagtccggaggcggaggcggacggatcgctcggctagaggaaaaagtgaaaaccttgaaagcgcaaaactccgagctggcgtccacggccaacatgctcagggaacaggtggcacagcttaagcagaaagtcatgaaccacgacaaaactcacacatgcccaccgtgcccagcacctgaactcctggggggaccgtcagtcttcctcttccccccaaaacccaaggacaccctcatgatctcccggacccctgaggtcacatgcgtggtggtggacgtgagccacgaagaccctgaggtcaagttcaactggtacgtggacggcgtggaggtgcataatgccaagacaaagccgcgggaggagcagtacaacagcacgtaccgtgtggtcagcgtcctcaccgtcctgcaccaggactggctgaatggcaaggagtacaagtgcaaggtctccaacaaagccctcccagcccccatcgagaaaaccatctccaaagccaaagggcagccccgagaaccacaggtgtacaccctgcccccatgccgggatgagctgaccaagaaccaggtcagcctgtggtgcctggtcaaaggcttctatcccagcgacatcgccgtggagtgggagagcaatgggcagccggagaacaactacaagaccacgcctcccgtgctggactccgacggctccttcttcctctacagcaagctcaccgtggacaagagtaggtggcagcaggggaacgtcttctcatgctccgtgatgcatgaggctctgcacaaccactacacacagaagagcctctccctgtctccgggcggctccggagccacgaacttctctctgttaaagcaagcaggagacgtggaagaaaaccccggtcccatggctatcatctacctcatcctcctgttcaccgctgtgcggggcgaagacgacattgaggccgaccacgtaggcttctatggtacaactgtttatcagtctcctggagacattggccagtacacacatgaatttgatggtgatgagttgttctatgtggacttggataagaagaaaactgtctggaggcttcctgagtttggccaattgatactctttgagccccaaggtggactgcaaaacatagctgcagaaaaacacaacttgggaatcttgactaagaggtcaaatttcaccccagctaccaatgaggctcctcaagcgactgtgttccccaagtcccctgtgctgctgggtcagcccaacacccttatctgctttgtggacaacatcttcccacctgtgatcaacatcacatggctcagaaatagcaagtcagtcacagacggcgtttatgagaccagcttcctcgtcaaccgtgaccattccttccacaagctgtcttatctcaccttcatcccttctgatgatgacatttatgactgcaaggtggagcactggggcctggaggagccggttctgaaacactgggaacctgagattccagcccccatgtcagagctgacagagtccggaggcggaggcggactgacagatacactccaagcggagacagatcaacttgaagacgagaagtctgcgttgcagaccgagattgccaatctactgaaagagaaggaaaaactggagtttattttggcagcccacgacaaaactcacacatgcccaccgtgcccagcacctgaactcctggggggaccgtcagtcttcctcttccccccaaaacccaaggacaccctcatgatctcccggacccctgaggtcacatgcgtggtggtggacgtgagccacgaagaccctgaggtcaagttcaactggtacgtggacggcgtggaggtgcataatgccaagacaaagccgcgggaggagcagtacaacagcacgtaccgtgtggtcagcgtcctcaccgtcctgcaccaggactggctgaatggcaaggagtacaagtgcaaggtctccaacaaagccctcccagcccccatcgagaaaaccatctccaaagccaaagggcagccccgagaaccacaggtgtgcaccctgcccccatcccgggatgagctgaccaagaaccaggtcagcctgagctgcgcggtcaaaggcttctatcccagcgacatcgccgtggagtgggagagcaatgggcagccggagaacaactacaagaccacgcctcccgtgctggactccgacggctccttcttcctcgtcagcaagctcaccgtggacaagagtaggtggcagcaggggaacgtcttctcatgctccgtgatgcatgaggctctgcacaaccactacacacagaagagcctctccctgtctcccggcggtagtggtagtggtagtggatctctgggtggtatcttcgaggctatgaagatggagctgcgcgatcaccatcaccatcaccataactggagccaccctcagttcgagaagtgt

SEQ ID NO: 8 - DNA, 2925 bp, Artificial Sequence
  source: /note="Description of Artificial Sequence: Synthetic polynucleotide"
atggctatcatctacctcatcctcctgttcaccgctgtgcggggcagatctgcccaccatcccatctgggcccgaatggacgccggaggtggaggctcactagtgccccgaggctctggaggtggaggctctggagactccgaaaggcatttcgtgcaccagttcaagggcgagtgctacttcaccaacgggacgcagcgcatacggctcgtgaccagatacatctacaaccgggaggagtacctgcgcttcgacagcgacgtgggcgagtaccgcgcggtgaccgagctggggcggcactcagccgagtactacaataagcagtacctggagcgaacgcgggccgagctggacacggcgtgcagacacaactacgaggagacggaggtccccacctccctgcggcggcttgaacagcccaatgtcgccatctccctgtccaggacagaggccctcaaccaccacaacactctggtctgttcggtgacagatttctacccagccaagatcaaagtgcgctggttcaggaatggccaggaggagacagtgggggtctcatccacacagcttattaggaatggggactggaccttccaggtcctggtcatgctggagatgacccctcatcagggagaggtctatacctgccatgtggagcatcccagcctgaagagccccatcactgtggagtggagggcacagtccgagtctgcccggagcaagtccggaggcggaggcggagacaaaactcacacatgcccaccgtgcccagcacctgaactcctggggggaccgtcagtcttcctcttccccccaaaacccaaggacaccctcatgatctcccggacccctgaggtcacatgcgtggtggtggacgtgagccacgaagaccctgaggtcaagttcaactggtacgtggacggcgtggaggtgcataatgccaagacaaagccgcgggaggagcagtacaacagcacgtaccgtgtggtcagcgtcctcaccgtcctgcaccaggactggctgaatggcaaggagtacaagtgcaaggtctccaacaaagccctcccagcccccatcgagaaaaccatctccaaagccaaagggcagccccgagaaccacaggtgtacaccctgcccccatgccgggatgagctgaccaagaaccaggtcagcctgtggtgcctggtcaaaggcttctatcccagcgacatcgccgtggagtgggagagcaatgggcagccggagaacaactacaagaccacgcctcccgtgctggactccgacggctccttcttcctctacagcaagctcaccgtggacaagagtaggtggcagcaggggaacgtcttctcatgctccgtgatgcatgaggctctgcacaaccactacacacagaagagcctctccctgtctccgggcggctccggagccacgaacttctctctgttaaagcaagcaggagacgtggaagaaaaccccggtcccatggctatcatctacctcatcctcctgttcaccgctgtgcggggcgaagacgacattgaggccgaccacgtaggcttctatggtacaactgtttatcagtctcctggagacattggccagtacacacatgaatttgatggtgatgagttgttctatgtggacttggataagaagaaaactgtctggaggcttcctgagtttggccaattgatactctttgagccccaaggtggactgcaaaacatagctgcagaaaaacacaacttgggaatcttgactaagaggtcaaatttcaccccagctaccaatgaggctcctcaagcgactgtgttccccaagtcccctgtgctgctgggtcagcccaacacccttatctgctttgtggacaacatcttcccacctgtgatcaacatcacatggctcagaaatagcaagtcagtcacagacggcgtttatgagaccagcttcctcgtcaaccgtgaccattccttccacaagctgtcttatctcaccttcatcccttctgatgatgacatttatgactgcaaggtggagcactggggcctggaggagccggttctgaaacactgggaacctgagattccagcccccatgtcagagctgacagagtccggaggcggaggcggagacaaaactcacacatgcccaccgtgcccagcacctgaactcctggggggaccgtcagtcttcctcttccccccaaaacccaaggacaccctcatgatctcccggacccctgaggtcacatgcgtggtggtggacgtgagccacgaagaccctgaggtcaagttcaactggtacgtggacggcgtggaggtgcataatgccaagacaaagccgcgggaggagcagtacaacagcacgtaccgtgtggtcagcgtcctcaccgtcctgcaccaggactggctgaatggcaaggagtacaagtgcaaggtctccaacaaagccctcccagcccccatcgagaaaaccatctccaaagccaaagggcagccccgagaaccacaggtgtgcaccctgcccccatcccgggatgagctgaccaagaaccaggtcagcctgagctgcgcggtcaaaggcttctatcccagcgacatcgccgtggagtgggagagcaatgggcagccggagaacaactacaagaccacgcctcccgtgctggactccgacggctccttcttcctcgtcagcaagctcaccgtggacaagagtaggtggcagcaggggaacgtcttctcatgctccgtgatgcatgaggctctgcacaaccactacacacagaagagcctctccctgtctcccggcggtagtggtagtggtagtggatctctgggtggtatcttcgaggctatgaagatggagctgcgcgatcaccatcaccatcaccataactggagccaccctcagttcgagaagtgt

SEQ ID NO: 9 - DNA, 1554 bp, Artificial Sequence
  source: /note="Description of Artificial Sequence: Synthetic polynucleotide"
atgggttctctgcaaccgctggccaccttgtacctgctgggtatgctggtcgctagcagcctcggacagcacctgcagaaggactacagagcctactacaccttcggaggtggaggcggctcaggaggtggaagcggcggctctggggacacccgaccacgtttcttggagtactctacgtctgagtgtcatttcttcaatgggacggagcgggtgcggtacctggacagatacttccataaccaggaggagaacgtgcgcttcgacagcgacgtgggggagttccgggcggtgacggagctggggcggcctgatgccgagtactggaacagccagaaggacctcctggagcagaagcggggccgggtggacaactactgcagacacaactacggggttgtggagagcttcacagtgcagcggcgagtccatcctaaggtgactgtgtatccttcaaagacccagcccctgcagcaccataacctcctggtctgttctgtgagtggtttctatccaggcagcattgaagtcaggtggttccggaatggccaggaagagaagactggggtggtgtccacaggcctgatccacaatggagactggaccttccagaccctggtgatgctggaaacagttcctcggagtggagaggtttacacctgccaagtggagcacccaagcgtgacaagccctctcacagtggaatggagagcacggtctgaatctgcacagagcaagtccggaggcggaggcggacggatcgctcggctagaggaaaaagtgaaaaccttgaaagcgcaaaactccgagctggcgtccacggccaacatgctcagggaacaggtggcacagcttaagcagaaagtcatgaaccacgacaaaactcacacatgcccaccgtgcccagcacctgaactcctggggggaccgtcagtcttcctcttccccccaaaacccaaggacaccctcatgatctcccggacccctgaggtcacatgcgtggtggtggacgtgagccacgaagaccctgaggtcaagttcaactggtacgtggacggcgtggaggtgcataatgccaagacaaagccgcgggaggagcagtacaacagcacgtaccgtgtggtcagcgtcctcaccgtcctgcaccaggactggctgaatggcaaggagtacaagtgcaaagtctccaacaaagccctcccagcccccatcgagaaaaccatctccaaagccaaagggcagccccgagaaccacaggtgtgcaccctgcccccatcccgggatgagctgaccaagaaccaggtcagcctgagctgcgcggtcaaaggcttctatcccagcgacatcgccgtggagtgggagagcaatgggcagccggagaacaactacaagaccacgcctcccgtgctggactccgacggctccttcttcctcgtcagcaagctcaccgtggacaagagcaggtggcagcaggggaacgtcttctcatgctccgtgatgcatgaggctctgcacaaccactacacacagaagagcctctccctgtctcccggc

SEQ ID NO: 10 - DNA, 1554 bp, Artificial Sequence
  source: /note="Description of Artificial Sequence: Synthetic polynucleotide"
atgggttctctgcaaccgctggccaccttgtacctgctgggtatgctggtcgctagcagcctcggacagcacctgcagaaggactacagagcctactacaccttcggaggtggaggcggctcaggaggtggaagcggcggctctggggacacccgaccacgtttcttggagtactctacgtctgagtgtcatttcttcaatgggacggagcgggtgcggtacctggacagatacttccataaccaggaggagaacgtgcgcttcgacagcgacgtgggggagttccgggcggtgacggagctggggcggcctgatgccgagtactggaacagccagaaggacctcctggagcagaagcggggccgggtggacaactactgcagacacaactacggggttgtggagagcttcacagtgcagcggcgagtccatcctaaggtgactgtgtatccttcaaagacccagcccctgcagcaccataacctcctggtctgttctgtgagtggtttctatccaggcagcattgaagtcaggtggttccggaatggccaggaagagaagactggggtggtgtccacaggcctgatccacaatggagactggaccttccagaccctggtgatgctggaaacagttcctcggagtggagaggtttacacctgccaagtggagcacccaagcgtgacaagccctctcacagtggaatggagagcacggtctgaatctgcacagagcaagtccggaggcggaggcggacggatcgctcggctagaggaaaaagtgaaaaccttgaaagcgcaaaactccgagctggcgtccacggccaacatgctcagggaacaggtggcacagcttaagcagaaagtcatgaaccacgacaaaactcacacatgcccaccgtgcccagcacctgaactcctggggggaccgtcagtcttcctcttccccccaaaacccaaggacaccctcatgatctcccggacccctgaggtcacatgcgtggtggtggacgtgagccacgaagaccctgaggtcaagttcaactggtacgtggacggcgtggaggtgcataatgccaagacaaagccgcgggaggagcagtacaacagcacgtaccgtgtggtcagcgtcctcaccgtcctgcaccaggactggctgaatggcaaggagtacaagtgcaaagtctccaacaaagccctcccagcccccatcgagaaaaccatctccaaagccaaagggcagccccgagaaccacaggtgtacaccctgcccccatgccgggatgagctgaccaagaaccaggtcagcctgtggtgcctggtcaaaggcttctatcccagcgacatcgccgtggagtgggagagcaatgggcagccggagaacaactacaagaccacgcctcccgtgctggactccgacggctccttcttcctctacagcaagctcaccgtggacaagagcaggtggcagcaggggaacgtcttctcatgctccgtgatgcatgaggctctgcacaaccactacacacagaagagcctctccctgtctccgggc

SEQ ID NO: 11 - DNA, 1434 bp, Artificial Sequence
  source: /note="Description of Artificial Sequence: Synthetic polynucleotide"
atggctatcatctacctcatcctcctgttcaccgctgtgcggggcatcaaagaagaacatgtgatcatccaggccgagttctatctgaatcctgaccaatcaggcgagtttatgtttgactttgatggtgatgagattttccatgtggatatggcaaagaaggagacggtctggcggcttgaagaatttggacgatttgccagctttgaggctcaaggtgcattggccaacatagctgtggacaaagccaacctggaaatcatgacaaagcgctccaactatactccgatcaccaatgtacctccagaggtaactgtgctcacaaacagccctgtggaactgagagagcccaacgtcctcatctgtttcatagacaagttcaccccaccagtggtcaatgtcacgtggcttcgaaatggaaaacctgtcaccacaggagtgtcagagacagtcttcctgcccagggaagaccaccttttccgcaagttccactatctccccttcctgccctcaactgaggacgtttacgactgcagggtggagcactggggcttggatgagcctcttctcaagcactgggagtttgatgctccaagccctctcccagagactacagagtccggaggcggaggcggactgacagatacactccaagcggagacagatcaacttgaagacgagaagtctgcgttgcagaccgagattgccaatctactgaaagagaaggaaaaactggagtttattttggcagcccacgacaaaactcacacatgcccaccgtgcccagcacctgaactcctggggggaccgtcagtcttcctcttccccccaaaacccaaggacaccctcatgatctcccggacccctgaggtcacatgcgtggtggtggacgtgagccacgaagaccctgaggtcaagttcaactggtacgtggacggcgtggaggtgcataatgccaagacaaagccgcgggaggagcagtacaacagcacgtaccgtgtggtcagcgtcctcaccgtcctgcaccaggactggctgaatggcaaggagtacaagtgcaaagtctccaacaaagccctcccagcccccatcgagaaaaccatctccaaagccaaagggcagccccgagaaccacaggtgtacaccctgcccccatgccgggatgagctgaccaagaaccaggtcagcctgtggtgcctggtcaaaggcttctatcccagcgacatcgccgtggagtgggagagcaatgggcagccggagaacaactacaagaccacgcctcccgtgctggactccgacggctccttcttcctctacagcaagctcaccgtggacaagagcaggtggcagcaggggaacgtcttctcatgctccgtgatgcatgaggctctgcacaaccactacacacagaagagcctctccctgtctccgggc

SEQ ID NO: 12 - DNA, 1434 bp, Artificial Sequence
  source: /note="Description of Artificial Sequence: Synthetic polynucleotide"
atggctatcatctacctcatcctcctgttcaccgctgtgcggggcatcaaagaagaacatgtgatcatccaggccgagttctatctgaatcctgaccaatcaggcgagtttatgtttgactttgatggtgatgagattttccatgtggatatggcaaagaaggagacggtctggcggcttgaagaatttggacgatttgccagctttgaggctcaaggtgcattggccaacatagctgtggacaaagccaacctggaaatcatgacaaagcgctccaactatactccgatcaccaatgtacctccagaggtaactgtgctcacaaacagccctgtggaactgagagagcccaacgtcctcatctgtttcatagacaagttcaccccaccagtggtcaatgtcacgtggcttcgaaatggaaaacctgtcaccacaggagtgtcagagacagtcttcctgcccagggaagaccaccttttccgcaagttccactatctccccttcctgccctcaactgaggacgtttacgactgcagggtggagcactggggcttggatgagcctcttctcaagcactgggagtttgatgctccaagccctctcccagagactacagagtccggaggcggaggcggactgacagatacactccaagcggagacagatcaacttgaagacgagaagtctgcgttgcagaccgagattgccaatctactgaaagagaaggaaaaactggagtttattttggcagcccacgacaaaactcacacatgcccaccgtgcccagcacctgaactcctggggggaccgtcagtcttcctcttccccccaaaacccaaggacaccctcatgatctcccggacccctgaggtcacatgcgtggtggtggacgtgagccacgaagaccctgaggtcaagttcaactggtacgtggacggcgtggaggtgcataatgccaagacaaagccgcgggaggagcagtacaacagcacgtaccgtgtggtcagcgtcctcaccgtcctgcaccaggactggctgaatggcaaggagtacaagtgcaaagtctccaacaaagccctcccagcccccatcgagaaaaccatctccaaagccaaagggcagccccgagaaccacaggtgtgcaccctgcccccatcccgggatgagctgaccaagaaccaggtcagcctgagctgcgcggtcaaaggcttctatcccagcgacatcgccgtggagtgggagagcaatgggcagccggagaacaactacaagaccacgcctcccgtgctggactccgacggctccttcttcctcgtcagcaagctcaccgtggacaagagcaggtggcagcaggggaacgtcttctcatgctccgtgatgcatgaggctctgcacaaccactacacacagaagagcctctccctgtctcccggc

SEQ ID NO: 13 - DNA, 1434 bp, Artificial Sequence
  source: /note="Description of Artificial Sequence: Synthetic polynucleotide"
atgggttctctgcaaccgctggccaccttgtacctgctgggtatgctggtcgctagcagcctcggacagcacctgcagaaggactacagagcctactacaccttcggaggtggaggcggctcaggaggtggaagcggcggctctggggacacccgaccacgtttcttggagtactctacgtctgagtgtcatttcttcaatgggacggagcgggtgcggtacctggacagatacttccataaccaggaggagaacgtgcgcttcgacagcgacgtgggggagttccgggcggtgacggagctggggcggcctgatgccgagtactggaacagccagaaggacctcctggagcagaagcggggccgggtggacaactactgcagacacaactacggggttgtggagagcttcacagtgcagcggcgagtccatcctaaggtgactgtgtatccttcaaagacccagcccctgcagcaccataacctcctggtctgttctgtgagtggtttctatccaggcagcattgaagtcaggtggttccggaatggccaggaagagaagactggggtggtgtccacaggcctgatccacaatggagactggaccttccagaccctggtgatgctggaaacagttcctcggagtggagaggtttacacctgccaagtggagcacccaagcgtgacaagccctctcacagtggaatggagagcacggtctgaatctgcacagagcaagtccggaggcggaggcggagacaaaactcacacatgcccaccgtgcccagcacctgaactcctggggggaccgtcagtcttcctcttccccccaaaacccaaggacaccctcatgatctcccggacccctgaggtcacatgcgtggtggtggacgtgagccacgaagaccctgaggtcaagttcaactggtacgtggacggcgtggaggtgcataatgccaagacaaagccgcgggaggagcagtacaacagcacgtaccgtgtggtcagcgtcctcaccgtcctgcaccaggactggctgaatggcaaggagtacaagtgcaaagtctccaacaaagccctcccagcccccatcgagaaaaccatctccaaagccaaagggcagccccgagaaccacaggtgtgcaccctgcccccatcccgggatgagctgaccaagaaccaggtcagcctgagctgcgcggtcaaaggcttctatcccagcgacatcgccgtggagtgggagagcaatgggcagccggagaacaactacaagaccacgcctcccgtgctggactccgacggctccttcttcctcgtcagcaagctcaccgtggacaagagcaggtggcagcaggggaacgtcttctcatgctccgtgatgcatgaggctctgcacaaccactacacacagaagagcctctccctgtctcccggc

SEQ ID NO: 14 - DNA, 1434 bp, Artificial Sequence
  source: /note="Description of Artificial Sequence: Synthetic polynucleotide"
atgggttctctgcaaccgctggccaccttgtacctgctgggtatgctggtcgctagcagcctcggacagcacctgcagaaggactacagagcctactacaccttcggaggtggaggcggctcaggaggtggaagcggcggctctggggacacccgaccacgtttcttggagtactctacgtctgagtgtcatttcttcaatgggacggagcgggtgcggtacctggacagatacttccataaccaggaggagaacgtgcgcttcgacagcgacgtgggggagttccgggcggtgacggagctggggcggcctgatgccgagtactggaacagccagaaggacctcctggagcagaagcggggccgggtggacaactactgcagacacaactacggggttgtggagagcttcacagtgcagcggcgagtccatcctaaggtgactgtgtatccttcaaagacccagcccctgcagcaccataacctcctggtctgttctgtgagtggtttctatccaggcagcattgaagtcaggtggttccggaatggccaggaagagaagactggggtggtgtccacaggcctgatccacaatggagactggaccttccagaccctggtgatgctggaaacagttcctcggagtggagaggtttacacctgccaagtggagcacccaagcgtgacaagccctctcacagtggaatggagagcacggtctgaatctgcacagagcaagtccggaggcggaggcggagacaaaactcacacatgcccaccgtgcccagcacctgaactcctggggggaccgtcagtcttcctcttccccccaaaacccaaggacaccctcatgatctcccggacccctgaggtcacatgcgtggtggtggacgtgagccacgaagaccctgaggtcaagttcaactggtacgtggacggcgtggaggtgcataatgccaagacaaagccgcgggaggagcagtacaacagcacgtaccgtgtggtcagcgtcctcaccgtcctgcaccaggactggctgaatggcaaggagtacaagtgcaaagtctccaacaaagccctcccagcccccatcgagaaaaccatctccaaagccaaagggcagccccgagaaccacaggtgtacaccctgcccccatgccgggatgagctgaccaagaaccaggtcagcctgtggtgcctggtcaaaggcttctatcccagcgacatcgccgtggagtgggagagcaatgggcagccggagaacaactacaagaccacgcctcccgtgctggactccgacggctccttcttcctctacagcaagctcaccgtggacaagagcaggtggcagcaggggaacgtcttctcatgctccgtgatgcatgaggctctgcacaaccactacacacagaagagcctctccctgtctccgggc

SEQ ID NO: 15 - DNA, 1314 bp, Artificial Sequence
  source: /note="Description of Artificial Sequence: Synthetic polynucleotide"
atggctatcatctacctcatcctcctgttcaccgctgtgcggggcatcaaagaagaacatgtgatcatccaggccgagttctatctgaatcctgaccaatcaggcgagtttatgtttgactttgatggtgatgagattttccatgtggatatggcaaagaaggagacggtctggcggcttgaagaatttggacgatttgccagctttgaggctcaaggtgcattggccaacatagctgtggacaaagccaacctggaaatcatgacaaagcgctccaactatactccgatcaccaatgtacctccagaggtaactgtgctcacaaacagccctgtggaactgagagagcccaacgtcctcatctgtttcatagacaagttcaccccaccagtggtcaatgtcacgtggcttcgaaatggaaaacctgtcaccacaggagtgtcagagacagtcttcctgcccagggaagaccaccttttccgcaagttccactatctccccttcctgccctcaactgaggacgtttacgactgcagggtggagcactggggcttggatgagcctcttctcaagcactgggagtttgatgctccaagccctctcccagagactacagagtccggaggcggaggcggagacaaaactcacacatgcccaccgtgcccagcacctgaactcctggggggaccgtcagtcttcctcttccccccaaaacccaaggacaccctcatgatctcccggacccctgaggtcacatgcgtggtggtggacgtgagccacgaagaccctgaggtcaagttcaactggtacgtggacggcgtggaggtgcataatgccaagacaaagccgcgggaggagcagtacaacagcacgtaccgtgtggtcagcgtcctcaccgtcctgcaccaggactggctgaatggcaaggagtacaagtgcaaagtctccaacaaagccctcccagcccccatcgagaaaaccatctccaaagccaaagggcagccccgagaaccacaggtgtacaccctgcccccatgccgggatgagctgaccaagaaccaggtcagcctgtggtgcctggtcaaaggcttctatcccagcgacatcgccgtggagtgggagagcaatgggcagccggagaacaactacaagaccacgcctcccgtgctggactccgacggctccttcttcctctacagcaagctcaccgtggacaagagcaggtggcagcaggggaacgtcttctcatgctccgtgatgcatgaggctctgcacaaccactacacacagaagagcctctccctgtctccgggc

SEQ ID NO: 16 - DNA, 1314 bp, Artificial Sequence
  source: /note="Description of Artificial Sequence: Synthetic polynucleotide"
atggctatcatctacctcatcctcctgttcaccgctgtgcggggcatcaaagaagaacatgtgatcatccaggccgagttctatctgaatcctgaccaatcaggcgagtttatgtttgactttgatggtgatgagattttccatgtggatatggcaaagaaggagacggtctggcggcttgaagaatttggacgatttgccagctttgaggctcaaggtgcattggccaacatagctgtggacaaagccaacctggaaatcatgacaaagcgctccaactatactccgatcaccaatgtacctccagaggtaactgtgctcacaaacagccctgtggaactgagagagcccaacgtcctcatctgtttcatagacaagttcaccccaccagtggtcaatgtcacgtggcttcgaaatggaaaacctgtcaccacaggagtgtcagagacagtcttcctgcccagggaagaccaccttttccgcaagttccactatctccccttcctgccctcaactgaggacgtttacgactgcagggtggagcactggggcttggatgagcctcttctcaagcactgggagtttgatgctccaagccctctcccagagactacagagtccggaggcggaggcggagacaaaactcacacatgcccaccgtgcccagcacctgaactcctggggggaccgtcagtcttcctcttccccccaaaacccaaggacaccctcatgatctcccggacccctgaggtcacatgcgtggtggtggacgtgagccacgaagaccctgaggtcaagttcaactggtacgtggacggcgtggaggtgcataatgccaagacaaagccgcgggaggagcagtacaacagcacgtaccgtgtggtcagcgtcctcaccgtcctgcaccaggactggctgaatggcaaggagtacaagtgcaaagtctccaacaaagccctcccagcccccatcgagaaaaccatctccaaagccaaagggcagccccgagaaccacaggtgtgcaccctgcccccatcccgggatgagctgaccaagaaccaggtcagcctgagctgcgcggtcaaaggcttctatcccagcgacatcgccgtggagtgggagagcaatgggcagccggagaacaactacaagaccacgcctcccgtgctggactccgacggctccttcttcctcgtcagcaagctcaccgtggacaagagcaggtggcagcaggggaacgtcttctcatgctccgtgatgcatgaggctctgcacaaccactacacacagaagagcctctccctgtctcccggc

SEQ ID NO: 17 - DNA, 1539 bp, Artificial Sequence
  source: /note="Description of Artificial Sequence: Synthetic polynucleotide"
atggctatcatctacctcatcctcctgttcaccgctgtgcggggcagatctgcccaccatcccatctgggcccgaatggacgccggaggtggaggctcactagtgccccgaggctctggaggtggaggctctggagactccgaaaggcatttcgtgcaccagttcaagggcgagtgctacttcaccaacgggacgcagcgcatacggctcgtgaccagatacatctacaaccgggaggagtacctgcgcttcgacagcgacgtgggcgagtaccgcgcggtgaccgagctggggcggcactcagccgagtactacaataagcagtacctggagcgaacgcgggccgagctggacacggcgtgcagacacaactacgaggagacggaggtccccacctccctgcggcggcttgaacagcccaatgtcgccatctccctgtccaggacagaggccctcaaccaccacaacactctggtctgttcggtgacagatttctacccagccaagatcaaagtgcgctggttcaggaatggccaggaggagacagtgggggtctcatccacacagcttattaggaatggggactggaccttccaggtcctggtcatgctggagatgacccctcatcagggagaggtctatacctgccatgtggagcatcccagcctgaagagccccatcactgtggagtggagggcacagtccgagtctgcccggagcaagtccggaggcggaggcggacggatcgctcggctagaggaaaaagtgaaaaccttgaaagcgcaaaactccgagctggcgtccacggccaacatgctcagggaacaggtggcacagcttaagcagaaagtcatgaaccacgacaaaactcacacatgcccaccgtgcccagcacctgaactcctggggggaccgtcagtcttcctcttccccccaaaacccaaggacaccctcatgatctcccggacccctgaggtcacatgcgtggtggtggacgtgagccacgaagaccctgaggtcaagttcaactggtacgtggacggcgtggaggtgcataatgccaagacaaagccgcgggaggagcagtacaacagcacgtaccgtgtggtcagcgtcctcaccgtcctgcaccaggactggctgaatggcaaggagtacaagtgcaaggtctccaacaaagccctcccagcccccatcgagaaaaccatctccaaagccaaagggcagccccgagaaccacaggtgtgcaccctgcccccatcccgggatgagctgaccaagaaccaggtcagcctgagctgcgcggtcaaaggcttctatcccagcgacatcgccgtggagtgggagagcaatgggcagccggagaacaactacaagaccacgcctcccgtgctggactccgacggctccttcttcctcgtcagcaagctcaccgtggacaagagtaggtggcagcaggggaacgtcttctcatgctccgtgatgcatgaggctctgcacaaccactacacacagaagagcctctccctgtctcccggc

SEQ ID NO: 18 - DNA, 1539 bp, Artificial Sequence
  source: /note="Description of Artificial Sequence: Synthetic polynucleotide"
atggctatcatctacctcatcctcctgttcaccgctgtgcggggcagatctgcccaccatcccatctgggcccgaatggacgccggaggtggaggctcactagtgccccgaggctctggaggtggaggctctggagactccgaaaggcatttcgtgcaccagttcaagggcgagtgctacttcaccaacgggacgcagcgcatacggctcgtgaccagatacatctacaaccgggaggagtacctgcgcttcgacagcgacgtgggcgagtaccgcgcggtgaccgagctggggcggcactcagccgagtactacaataagcagtacctggagcgaacgcgggccgagctggacacggcgtgcagacacaactacgaggagacggaggtccccacctccctgcggcggcttgaacagcccaatgtcgccatctccctgtccaggacagaggccctcaaccaccacaacactctggtctgttcggtgacagatttctacccagccaagatcaaagtgcgctggttcaggaatggccaggaggagacagtgggggtctcatccacacagcttattaggaatggggactggaccttccaggtcctggtcatgctggagatgacccctcatcagggagaggtctatacctgccatgtggagcatcccagcctgaagagccccatcactgtggagtggagggcacagtccgagtctgcccggagcaagtccggaggcggaggcggacggatcgctcggctagaggaaaaagtgaaaaccttgaaagcgcaaaactccgagctggcgtccacggccaacatgctcagggaacaggtggcacagcttaagcagaaagtcatgaaccacgacaaaactcacacatgcccaccgtgcccagcacctgaactcctggggggaccgtcagtcttcctcttccccccaaaacccaaggacaccctcatgatctcccggacccctgaggtcacatgcgtggtggtggacgtgagccacgaagaccctgaggtcaagttcaactggtacgtggacggcgtggaggtgcataatgccaagacaaagccgcgggaggagcagtacaacagcacgtaccgtgtggtcagcgtcctcaccgtcctgcaccaggactggctgaatggcaaggagtacaagtgcaaggtctccaacaaagccctcccagcccccatcgagaaaaccatctccaaagccaaagggcagccccgagaaccacaggtgtacaccctgcccccatgccgggatgagctgaccaagaaccaggtcagcctgtggtgcctggtcaaaggcttctatcccagcgacatcgccgtggagtgggagagcaatgggcagccggagaacaactacaagaccacgcctcccgtgctggactccgacggctccttcttcctctacagcaagctcaccgtggacaagagtaggtggcagcaggggaacgtcttctcatgctccgtgatgcatgaggctctgcacaaccactacacacagaagagcctctccctgtctccgggc

SEQ ID NO: 19 - DNA, 1446 bp, Artificial Sequence
  source: /note="Description of Artificial Sequence: Synthetic polynucleotide"
atggctatcatctacctcatcctcctgttcaccgctgtgcggggcgaagacgacattgaggccgaccacgtaggcttctatggtacaactgtttatcagtctcctggagacattggccagtacacacatgaatttgatggtgatgagttgttctatgtggacttggataagaagaaaactgtctggaggcttcctgagtttggccaattgatactctttgagccccaaggtggactgcaaaacatagctgcagaaaaacacaacttgggaatcttgactaagaggtcaaatttcaccccagctaccaatgaggctcctcaagcgactgtgttccccaagtcccctgtgctgctgggtcagcccaacacccttatctgctttgtggacaacatcttcccacctgtgatcaacatcacatggctcagaaatagcaagtcagtcacagacggcgtttatgagaccagcttcctcgtcaaccgtgaccattccttccacaagctgtcttatctcaccttcatcccttctgatgatgacatttatgactgcaaggtggagcactggggcctggaggagccggttctgaaacactgggaacctgagattccagcccccatgtcagagctgacagagtccggaggcggaggcggactgacagatacactccaagcggagacagatcaacttgaagacgagaagtctgcgttgcagaccgagattgccaatctactgaaagagaaggaaaaactggagtttattttggcagcccacgacaaaactcacacatgcccaccgtgcccagcacctgaactcctggggggaccgtcagtcttcctcttccccccaaaacccaaggacaccctcatgatctcccggacccctgaggtcacatgcgtggtggtggacgtgagccacgaagaccctgaggtcaagttcaactggtacgtggacggcgtggaggtgcataatgccaagacaaagccgcgggaggagcagtacaacagcacgtaccgtgtggtcagcgtcctcaccgtcctgcaccaggactggctgaatggcaaggagtacaagtgcaaggtctccaacaaagccctcccagcccccatcgagaaaaccatctccaaagccaaagggcagccccgagaaccacaggtgtacaccctgcccccatgccgggatgagctgaccaagaaccaggtcagcctgtggtgcctggtcaaaggcttctatcccagcgacatcgccgtggagtgggagagcaatgggcagccggagaacaactacaagaccacgcctcccgtgctggactccgacggctccttcttcctctacagcaagctcaccgtggacaagagtaggtggcagcaggggaacgtcttctcatgctccgtgatgcatgaggctctgcacaaccactacacacagaagagcctctccctgtctccgggc

SEQ ID NO: 20 - DNA, 1446 bp, Artificial Sequence
  source: /note="Description of Artificial Sequence: Synthetic polynucleotide"
atggctatcatctacctcatcctcctgttcaccgctgtgcggggcgaagacgacattgaggccgaccacgtaggcttctatggtacaactgtttatcagtctcctggagacattggccagtacacacatgaatttgatggtgatgagttgttctatgtggacttggataagaagaaaactgtctggaggcttcctgagtttggccaattgatactctttgagccccaaggtggactgcaaaacatagctgcagaaaaacacaacttgggaatcttgactaagaggtcaaatttcaccccagctaccaatgaggctcctcaagcgactgtgttccccaagtcccctgtgctgctgggtcagcccaacacccttatctgctttgtggacaacatcttcccacctgtgatcaacatcacatggctcagaaatagcaagtcagtcacagacggcgtttatgagaccagcttcctcgtcaaccgtgaccattccttccacaagctgtcttatctcaccttcatcccttctgatgatgacatttatgactgcaaggtggagcactggggcctggaggagccggttctgaaacactgggaacctgagattccagcccccatgtcagagctgacagagtccggaggcggaggcggactgacagatacactccaagcggagacagatcaacttgaagacgagaagtctgcgttgcagaccgagattgccaatctactgaaagagaaggaaaaactggagtttattttggcagcccacgacaaaactcacacatgcccaccgtgcccagcacctgaactcctggggggaccgtcagtcttcctcttccccccaaaacccaaggacaccctcatgatctcccggacccctgaggtcacatgcgtggtggtggacgtgagccacgaagaccctgaggtcaagttcaactggtacgtggacggcgtggaggtgcataatgccaagacaaagccgcgggaggagcagtacaacagcacgtaccgtgtggtcagcgtcctcaccgtcctgcaccaggactggctgaatggcaaggagtacaagtgcaaggtctccaacaaagccctcccagcccccatcgagaaaaccatctccaaagccaaagggcagccccgagaaccacaggtgtgcaccctgcccccatcccgggatgagctgaccaagaaccaggtcagcctgagctgcgcggtcaaaggcttctatcccagcgacatcgccgtggagtgggagagcaatgggcagccggagaacaactacaagaccacgcctcccgtgctggactccgacggctccttcttcctcgtcagcaagctcaccgtggacaagagtaggtggcagcaggggaacgtcttctcatgctccgtgatgcatgaggctctgcacaaccactacacacagaagagcctctccctgtctcccggc

SEQ ID NO: 21 - DNA, 1419 bp, Artificial Sequence
  source: /note="Description of Artificial Sequence: Synthetic polynucleotide"
atggctatcatctacctcatcctcctgttcaccgctgtgcggggcagatctgcccaccatcccatctgggcccgaatggacgccggaggtggaggctcactagtgccccgaggctctggaggtggaggctctggagactccgaaaggcatttcgtgcaccagttcaagggcgagtgctacttcaccaacgggacgcagcgcatacggctcgtgaccagatacatctacaaccgggaggagtacctgcgcttcgacagcgacgtgggcgagtaccgcgcggtgaccgagctggggcggcactcagccgagtactacaataagcagtacctggagcgaacgcgggccgagctggacacggcgtgcagacacaactacgaggagacggaggtccccacctccctgcggcggcttgaacagcccaatgtcgccatctccctgtccaggacagaggccctcaaccaccacaacactctggtctgttcggtgacagatttctacccagccaagatcaaagtgcgctggttcaggaatggccaggaggagacagtgggggtctcatccacacagcttattaggaatggggactggaccttccaggtcctggtcatgctggagatgacccctcatcagggagaggtctatacctgccatgtggagcatcccagcctgaagagccccatcactgtggagtggagggcacagtccgagtctgcccggagcaagtccggaggcggaggcggagacaaaactcacacatgcccaccgtgcccagcacctgaactcctggggggaccgtcagtcttcctcttccccccaaaacccaaggacaccctcatgatctcccggacccctgaggtcacatgcgtggtggtggacgtgagccacgaagaccctgaggtcaagttcaactggtacgtggacggcgtggaggtgcataatgccaagacaaagccgcgggaggagcagtacaacagcacgtaccgtgtggtcagcgtcctcaccgtcctgcaccaggactggctgaatggcaaggagtacaagtgcaaggtctccaacaaagccctcccagcccccatcgagaaaaccatctccaaagccaaagggcagccccgagaaccacaggtgtgcaccctgcccccatcccgggatgagctgaccaagaaccaggtcagcctgagctgcgcggtcaaaggcttctatcccagcgacatcgccgtggagtgggagagcaatgggcagccggagaacaactacaagaccacgcctcccgtgctggactccgacggctccttcttcctcgtcagcaagctcaccgtggacaagagtaggtggcagcaggggaacgtcttctcatgctccgtgatgcatgaggctctgcacaaccactacacacagaagagcctctccctgtctcccggc

SEQ ID NO: 22 - DNA, 1419 bp, Artificial Sequence
  source: /note="Description of Artificial Sequence: Synthetic polynucleotide"
atggctatcatctacctcatcctcctgttcaccgctgtgcggggcagatctgcccaccatcccatctgggcccgaatggacgccggaggtggaggctcactagtgccccgaggctctggaggtggaggctctggagactccgaaaggcatttcgtgcaccagttcaagggcgagtgctacttcaccaacgggacgcagcgcatacggctcgtgaccagatacatctacaaccgggaggagtacctgcgcttcgacagcgacgtgggcgagtaccgcgcggtgaccgagctggggcggcactcagccgagtactacaataagcagtacctggagcgaacgcgggccgagctggacacggcgtgcagacacaactacgaggagacggaggtccccacctccctgcggcggcttgaacagcccaatgtcgccatctccctgtccaggacagaggccctcaaccaccacaacactctggtctgttcggtgacagatttctacccagccaagatcaaagtgcgctggttcaggaatggccaggaggagacagtgggggtctcatccacacagcttattaggaatggggactggaccttccaggtcctggtcatgctggagatgacccctcatcagggagaggtctatacctgccatgtggagcatcccagcctgaagagccccatcactgtggagtggagggcacagtccgagtctgcccggagcaagtccggaggcggaggcggagacaaaactcacacatgcccaccgtgcccagcacctgaactcctggggggaccgtcagtcttcctcttccccccaaaacccaaggacaccctcatgatctcccggacccctgaggtcacatgcgtggtggtggacgtgagccacgaagaccctgaggtcaagttcaactggtacgtggacggcgtggaggtgcataatgccaagacaaagccgcgggaggagcagtacaacagcacgtaccgtgtggtcagcgtcctcaccgtcctgcaccaggactggctgaatggcaaggagtacaagtgcaaggtctccaacaaagccctcccagcccccatcgagaaaaccatctccaaagccaaagggcagccccgagaaccacaggtgtacaccctgcccccatgccgggatgagctgaccaagaaccaggtcagcctgtggtgcctggtcaaaggcttctatcccagcgacatcgccgtggagtgggagagcaatgggcagccggagaacaactacaagaccacgcctcccgtgctggactccgacggctccttcttcctctacagcaagctcaccgtggacaagagtaggtggcagcaggggaacgtcttctcatgctccgtgatgcatgaggctctgcacaaccactacacacagaagagcctctccctgtctccgggc

SEQ ID NO: 23 - DNA, 1326 bp, Artificial Sequence
  source: /note="Description of Artificial Sequence: Synthetic polynucleotide"
atggctatcatctacctcatcctcctgttcaccgctgtgcggggcgaagacgacattgaggccgaccacgtaggcttctatggtacaactgtttatcagtctcctggagacattggccagtacacacatgaatttgatggtgatgagttgttctatgtggacttggataagaagaaaactgtctggaggcttcctgagtttggccaattgatactctttgagccccaaggtggactgcaaaacatagctgcagaaaaacacaacttgggaatcttgactaagaggtcaaatttcaccccagctaccaatgaggctcctcaagcgactgtgttccccaagtcccctgtgctgctgggtcagcccaacacccttatctgctttgtggacaacatcttcccacctgtgatcaacatcacatggctcagaaatagcaagtcagtcacagacggcgtttatgagaccagcttcctcgtcaaccgtgaccattccttccacaagctgtcttatctcaccttcatcccttctgatgatgacatttatgactgcaaggtggagcactggggcctggaggagccggttctgaaacactgggaacctgagattccagcccccatgtcagagctgacagagtccggaggcggaggcggagacaaaactcacacatgcccaccgtgcccagcacctgaactcctggggggaccgtcagtcttcctcttccccccaaaacccaaggacaccctcatgatctcccggacccctgaggtcacatgcgtggtggtggacgtgagccacgaagaccctgaggtcaagttcaactggtacgtggacggcgtggaggtgcataatgccaagacaaagccgcgggaggagcagtacaacagcacgtaccgtgtggtcagcgtcctcaccgtcctgcaccaggactggctgaatggcaaggagtacaagtgcaaggtctccaacaaagccctcccagcccccatcgagaaaaccatctccaaagccaaagggcagccccgagaaccacaggtgtacaccctgcccccatgccgggatgagctgaccaagaaccaggtcagcctgtggtgcctggtcaaaggcttctatcccagcgacatcgccgtggagtgggagagcaatgggcagccggagaacaactacaagaccacgcctcccgtgctggactccgacggctccttcttcctctacagcaagctcaccgtggacaagagtaggtggcagcaggggaacgtcttctcatgctccgtgatgcatgaggctctgcacaaccactacacacagaagagcctctccctgtctccgggc

SEQ ID NO: 24 - DNA, 1326 bp, Artificial Sequence
  source: /note="Description of Artificial Sequence: Synthetic polynucleotide"
atggctatcatctacctcatcctcctgttcaccgctgtgcggggcgaagacgacattgaggccgaccacgtaggcttctatggtacaactgtttatcagtctcctggagacattggccagtacacacatgaatttgatggtgatgagttgttctatgtggacttggataagaagaaaactgtctggaggcttcctgagtttggccaattgatactctttgagccccaaggtggactgcaaaacatagctgcagaaaaacacaacttgggaatcttgactaagaggtcaaatttcaccccagctaccaatgaggctcctcaagcgactgtgttccccaagtcccctgtgctgctgggtcagcccaacacccttatctgctttgtggacaacatcttcccacctgtgatcaacatcacatggctcagaaatagcaagtcagtcacagacggcgtttatgagaccagcttcctcgtcaaccgtgaccattccttccacaagctgtcttatctcaccttcatcccttctgatgatgacatttatgactgcaaggtggagcactggggcctggaggagccggttctgaaacactgggaacctgagattccagcccccatgtcagagctgacagagtccggaggcggaggcggagacaaaactcacacatgcccaccgtgcccagcacctgaactcctggggggaccgtcagtcttcctcttccccccaaaacccaaggacaccctcatgatctcccggacccctgaggtcacatgcgtggtggtggacgtgagccacgaagaccctgaggtcaagttcaactggtacgtggacggcgtggaggtgcataatgccaagacaaagccgcgggaggagcagtacaacagcacgtaccgtgtggtcagcgtcctcaccgtcctgcaccaggactggctgaatggcaaggagtacaagtgcaaggtctccaacaaagccctcccagcccccatcgagaaaaccatctccaaagccaaagggcagccccgagaaccacaggtgtgcaccctgcccccatcccgggatgagctgaccaagaaccaggtcagcctgagctgcgcggtcaaaggcttctatcccagcgacatcgccgtggagtgggagagcaatgggcagccggagaacaactacaagaccacgcctcccgtgctggactccgacggctccttcttcctcgtcagcaagctcaccgtggacaagagtaggtggcagcaggggaacgtcttctcatgctccgtgatgcatgaggctctgcacaaccactacacacagaagagcctctccctgtctcccggc

SEQ ID NO: 25 - DNA, 678 bp, Artificial Sequence
  source: /note="Description of Artificial Sequence: Synthetic polynucleotide"
gacaaaactcacacatgcccaccgtgcccagcacctgaactcctggggggaccgtcagtcttcctcttccccccaaaacccaaggacaccctcatgatctcccggacccctgaggtcacatgcgtggtggtggacgtgagccacgaagaccctgaggtcaagttcaactggtacgtggacggcgtggaggtgcataatgccaagacaaagccgcgggaggagcagtacaacagcacgtaccgtgtggtcagcgtcctcaccgtcctgcaccaggactggctgaatggcaaggagtacaagtgcaaagtctccaacaaagccctcccagcccccatcgagaaaaccatctccaaagccaaagggcagccccgagaaccacaggtgtgcaccctgcccccatcccgggatgagctgaccaagaaccaggtcagcctgagctgcgcggtcaaaggcttctatcccagcgacatcgccgtggagtgggagagcaatgggcagccggagaacaactacaagaccacgcctcccgtgctggactccgacggctccttcttcctcgtcagcaagctcaccgtggacaagagcaggtggcagcaggggaacgtcttctcatgctccgtgatgcatgaggctctgcacaaccactacacacagaagagcctctccctgtctcccggc

SEQ ID NO: 26 - DNA, 678 bp, Artificial Sequence
  source: /note="Description of Artificial Sequence: Synthetic polynucleotide"
gacaaaactcacacatgcccaccgtgcccagcacctgaactcctggggggaccgtcagtcttcctcttccccccaaaacccaaggacaccctcatgatctcccggacccctgaggtcacatgcgtggtggtggacgtgagccacgaagaccctgaggtcaagttcaactggtacgtggacggcgtggaggtgcataatgccaagacaaagccgcgggaggagcagtacaacagcacgtaccgtgtggtcagcgtcctcaccgtcctgcaccaggactggctgaatggcaaggagtacaagtgcaaagtctccaacaaagccctcccagcccccatcgagaaaaccatctccaaagccaaagggcagccccgagaaccacaggtgtacaccctgcccccatgccgggatgagctgaccaagaaccaggtcagcctgtggtgcctggtcaaaggcttctatcccagcgacatcgccgtggagtgggagagcaatgggcagccggagaacaactacaagaccacgcctcccgtgctggactccgacggctccttcttcctctacagcaagctcaccgtggacaagagcaggtggcagcaggggaacgtcttctcatgctccgtgatgcatgaggctctgcacaaccactacacacagaagagcctctccctgtctccgggc

SEQ ID NO: 27 - protein, 1056 aa, Artificial Sequence
  source: /note="Description of Artificial Sequence: Synthetic polypeptide"
MGSLQPLATLYLLGMLVASSLGQHLQKDYRAYYTFGGGGGSGGGSGGSGDTRPRFLEYSTSECHFFNGTERVRYLDRYFHNQEENVRFDSDVGEFRAVTELGRPDAEYWNSQKDLLEQKRGRVDNYCRHNYGVVESFTVQRRVHPKVTVYPSKTQPLQHHNLLVCSVSGFYPGSIEVRWFRNGQEEKTGVVSTGLIHNGDWTFQTLVMLETVPRSGEVYTCQVEHPSVTSPLTVEWRARSESAQSKSGGGGGRIARLEEKVKTLKAQNSELASTANMLREQVAQLKQKVMNHDKTHTCPPCPAPELLGGPSVFLFPPKPKDTLMISRTPEVTCVVVDVSHEDPEVKFNWYVDGVEVHNAKTKPREEQYNSTYRVVSVLTVLHQDWLNGKEYKCKVSNKALPAPIEKTISKAKGQPREPQVCTLPPSRDELTKNQVSLSCAVKGFYPSDIAVEWESNGQPENNYKTTPPVLDSDGSFFLVSKLTVDKSRWQQGNVFSCSVMHEALHNHYTQKSLSLSPGGSGATNFSLLKQAGDVEENPGPMAIIYLILLFTAVRGIKEEHVIIQAEFYLNPDQSGEFMFDFDGDEIFHVDMAKKETVWRLEEFGRFASFEAQGALANIAVDKANLEIMTKRSNYTPITNVPPEVTVLTNSPVELREPNVLICFIDKFTPPVVNVTWLRNGKPVTTGVSETVFLPREDHLFRKFHYLPFLPSTEDVYDCRVEHWGLDEPLLKHWEFDAPSPLPETTESGGGGGLTDTLQAETDQLEDEKSALQTEIANLLKEKEKLEFILAAHDKTHTCPPCPAPELLGGPSVFLFPPKPKDTLMISRTPEVTCVVVDVSHEDPEVKFNWYVDGVEVHNAKTKPREEQYNSTYRVVSVLTVLHQDWLNGKEYKCKVSNKALPAPIEKTISKAKGQPREPQVYTLPPCRDELTKNQVSLWCLVKGFYPSDIAVEWESNGQPENNYKTTPPVLDSDGSFFLYSKLTVDKSRWQQGNVFSCSVMHEALHNHYTQKSLSLSPGGSGSGSGSLGGIFEAMKMELRDHHHHHHNWSHPQFEKC

SEQ ID NO: 28 - protein, 976 aa, Artificial Sequence
  source: /note="Description of Artificial Sequence: Synthetic polypeptide"
MGSLQPLATLYLLGMLVASSLGQHLQKDYRAYYTFGGGGGSGGGSGGSGDTRPRFLEYSTSECHFFNGTERVRYLDRYFHNQEENVRFDSDVGEFRAVTELGRPDAEYWNSQKDLLEQKRGRVDNYCRHNYGVVESFTVQRRVHPKVTVYPSKTQPLQHHNLLVCSVSGFYPGSIEVRWFRNGQEEKTGVVSTGLIHNGDWTFQTLVMLETVPRSGEVYTCQVEHPSVTSPLTVEWRARSESAQSKSGGGGGDKTHTCPPCPAPELLGGPSVFLFPPKPKDTLMISRTPEVTCVVVDVSHEDPEVKFNWYVDGVEVHNAKTKPREEQYNSTYRVVSVLTVLHQDWLNGKEYKCKVSNKALPAPIEKTISKAKGQPREPQVCTLPPSRDELTKNQVSLSCAVKGFYPSDIAVEWESNGQPENNYKTTPPVLDSDGSFFLVSKLTVDKSRWQQGNVFSCSVMHEALHNHYTQKSLSLSPGGSGATNFSLLKQAGDVEENPGPMAIIYLILLFTAVRGIKEEHVIIQAEFYLNPDQSGEFMFDFDGDEIFHVDMAKKETVWRLEEFGRFASFEAQGALANIAVDKANLEIMTKRSNYTPITNVPPEVTVLTNSPVELREPNVLICFIDKFTPPVVNVTWLRNGKPVTTGVSETVFLPREDHLFRKFHYLPFLPSTEDVYDCRVEHWGLDEPLLKHWEFDAPSPLPETTESGGGGGDKTHTCPPCPAPELLGGPSVFLFPPKPKDTLMISRTPEVTCVVVDVSHEDPEVKFNWYVDGVEVHNAKTKPREEQYNSTYRVVSVLTVLHQDWLNGKEYKCKVSNKALPAPIEKTISKAKGQPREPQVYTLPPCRDELTKNQVSLWCLVKGFYPSDIAVEWESNGQPENNYKTTPPVLDSDGSFFLYSKLTVDKSRWQQGNVFSCSVMHEALHNHYTQKSLSLSPGGSGSGSGSLGGIFEAMKMELRDHHHHHHNWSHPQFEKC

SEQ ID NO: 29 - protein, 1055 aa, Artificial Sequence
  source: /note="Description of Artificial Sequence: Synthetic polypeptide"
MAIIYLILLFTAVRGRSAHHPIWARMDAGGGGSLVPRGSGGGGSGDSERHFVHQFKGECYFTNGTQRIRLVTRYIYNREEYLRFDSDVGEYRAVTELGRHSAEYYNKQYLERTRAELDTACRHNYEETEVPTSLRRLEQPNVAISLSRTEALNHHNTLVCSVTDFYPAKIKVRWFRNGQEETVGVSSTQLIRNGDWTFQVLVMLEMTPHQGEVYTCHVEHPSLKSPITVEWRAQSESARSKSGGGGGRIARLEEKVKTLKAQNSELASTANMLREQVAQLKQKVMNHDKTHTCPPCPAPELLGGPSVFLFPPKPKDTLMISRTPEVTCVVVDVSHEDPEVKFNWYVDGVEVHNAKTKPREEQYNSTYRVVSVLTVLHQDWLNGKEYKCKVSNKALPAPIEKTISKAKGQPREPQVCTLPPSRDELTKNQVSLSCAVKGFYPSDIAVEWESNGQPENNYKTTPPVLDSDGSFFLVSKLTVDKSRWQQGNVFSCSVMHEALHNHYTQKSLSLSPGGSGATNFSLLKQAGDVEENPGPMAIIYLILLFTAVRGEDDIEADHVGFYGTTVYQSPGDIGQYTHEFDGDELFYVDLDKKKTVWRLPEFGQLILFEPQGGLQNIAAEKHNLGILTKRSNFTPATNEAPQATVFPKSPVLLGQPNTLICFVDNIFPPVINITWLRNSKSVTDGVYETSFLVNRDHSFHKLSYLTFIPSDDDIYDCKVEHWGLEEPVLKHWEPEIPAPMSELTESGGGGGLTDTLQAETDQLEDEKSALQTEIANLLKEKEKLEFILAAHDKTHTCPPCPAPELLGGPSVFLFPPKPKDTLMISRTPEVTCVVVDVSHEDPEVKFNWYVDGVEVHNAKTKPREEQYNSTYRVVSVLTVLHQDWLNGKEYKCKVSNKALPAPIEKTISKAKGQPREPQVYTLPPCRDELTKNQVSLWCLVKGFYPSDIAVEWESNGQPENNYKTTPPVLDSDGSFFLYSKLTVDKSRWQQGNVFSCSVMHEALHNHYTQKSLSLSPGGSGSGSGSLGGIFEAMKMELRDHHHHHHNWSHPQFEKC

SEQ ID NO: 30 - protein, 975 aa, Artificial Sequence
  source: /note="Description of Artificial Sequence: Synthetic polypeptide"
MAIIYLILLFTAVRGRSAHHPIWARMDAGGGGSLVPRGSGGGGSGDSERHFVHQFKGECYFTNGTQRIRLVTRYIYNREEYLRFDSDVGEYRAVTELGRHSAEYYNKQYLERTRAELDTACRHNYEETEVPTSLRRLEQPNVAISLSRTEALNHHNTLVCSVTDFYPAKIKVRWFRNGQEETVGVSSTQLIRNGDWTFQVLVMLEMTPHQGEVYTCHVEHPSLKSPITVEWRAQSESARSKSGGGGGDKTHTCPPCPAPELLGGPSVFLFPPKPKDTLMISRTPEVTCVVVDVSHEDPEVKFNWYVDGVEVHNAKTKPREEQYNSTYRVVSVLTVLHQDWLNGKEYKCKVSNKALPAPIEKTISKAKGQPREPQVCTLPPSRDELTKNQVSLSCAVKGFYPSDIAVEWESNGQPENNYKTTPPVLDSDGSFFLVSKLTVDKSRWQQGNVFSCSVMHEALHNHYTQKSLSLSPGGSGATNFSLLKQAGDVEENPGPMAIIYLILLFTAVRGEDDIEADHVGFYGTTVYQSPGDIGQYTHEFDGDELFYVDLDKKKTVWRLPEFGQLILFEPQGGLQNIAAEKHNLGILTKRSNFTPATNEAPQATVFPKSPVLLGQPNTLICFVDNIFPPVINITWLRNSKSVTDGVYETSFLVNRDHSFHKLSYLTFIPSDDDIYDCKVEHWGLEEPVLKHWEPEIPAPMSELTESGGGGGDKTHTCPPCPAPELLGGPSVFLFPPKPKDTLMISRTPEVTCVVVDVSHEDPEVKFNWYVDGVEVHNAKTKPREEQYNSTYRVVSVLTVLHQDWLNGKEYKCKVSNKALPAPIEKTISKAKGQPREPQVYTLPPCRDELTKNQVSLWCLVKGFYPSDIAVEWESNGQPENNYKTTPPVLDSDGSFFLYSKLTVDKSRWQQGNVFSCSVMHEALHNHYTQKSLSLSPGGSGSGSGSLGGIFEAMKMELRDHHHHHHNWSHPQFEKC

SEQ ID NO: 31 - protein, 1056 aa, Artificial Sequence
  source: /note="Description of Artificial Sequence: Synthetic polypeptide"
MGSLQPLATLYLLGMLVASSLGQHLQKDYRAYYTFGGGGGSGGGSGGSGDTRPRFLEYSTSECHFFNGTERVRYLDRYFHNQEENVRFDSDVGEFRAVTELGRPDAEYWNSQKDLLEQKRGRVDNYCRHNYGVVESFTVQRRVHPKVTVYPSKTQPLQHHNLLVCSVSGFYPGSIEVRWFRNGQEEKTGVVSTGLIHNGDWTFQTLVMLETVPRSGEVYTCQVEHPSVTSPLTVEWRARSESAQSKSGGGGGRIARLEEKVKTLKAQNSELASTANMLREQVAQLKQKVMNHDKTHTCPPCPAPELLGGPSVFLFPPKPKDTLMISRTPEVTCVVVDVSHEDPEVKFNWYVDGVEVHNAKTKPREEQYNSTYRVVSVLTVLHQDWLNGKEYKCKVSNKALPAPIEKTISKAKGQPREPQVYTLPPCRDELTKNQVSLWCLVKGFYPSDIAVEWESNGQPENNYKTTPPVLDSDGSFFLYSKLTVDKSRWQQGNVFSCSVMHEALHNHYTQKSLSLSPGGSGATNFSLLKQAGDVEENPGPMAIIYLILLFTAVRGIKEEHVIIQAEFYLNPDQSGEFMFDFDGDEIFHVDMAKKETVWRLEEFGRFASFEAQGALANIAVDKANLEIMTKRSNYTPITNVPPEVTVLTNSPVELREPNVLICFIDKFTPPVVNVTWLRNGKPVTTGVSETVFLPREDHLFRKFHYLPFLPSTEDVYDCRVEHWGLDEPLLKHWEFDAPSPLPETTESGGGGGLTDTLQAETDQLEDEKSALQTEIANLLKEKEKLEFILAAHDKTHTCPPCPAPELLGGPSVFLFPPKPKDTLMISRTPEVTCVVVDVSHEDPEVKFNWYVDGVEVHNAKTKPREEQYNSTYRVVSVLTVLHQDWLNGKEYKCKVSNKALPAPIEKTISKAKGQPREPQVCTLPPSRDELTKNQVSLSCAVKGFYPSDIAVEWESNGQPENNYKTTPPVLDSDGSFFLVSKLTVDKSRWQQGNVFSCSVMHEALHNHYTQKSLSLSPGGSGSGSGSLGGIFEAMKMELRDHHHHHHNWSHPQFEKC

SEQ ID NO: 32 - protein, 976 aa, Artificial Sequence
  source: /note="Description of Artificial Sequence: Synthetic polypeptide"
MGSLQPLATLYLLGMLVASSLGQHLQKDYRAYYTFGGGGGSGGGSGGSGDTRPRFLEYSTSECHFFNGTERVRYLDRYFHNQEENVRFDSDVGEFRAVTELGRPDAEYWNSQKDLLEQKRGRVDNYCRHNYGVVESFTVQRRVHPKVTVYPSKTQPLQHHNLLVCSVSGFYPGSIEVRWFRNGQEEKTGVVSTGLIHNGDWTFQTLVMLETVPRSGEVYTCQVEHPSVTSPLTVEWRARSESAQSKSGGGGGDKTHTCPPCPAPELLGGPSVFLFPPKPKDTLMISRTPEVTCVVVDVSHEDPEVKFNWYVDGVEVHNAKTKPREEQYNSTYRVVSVLTVLHQDWLNGKEYKCKVSNKALPAPIEKTISKAKGQPREPQVYTLPPCRDELTKNQVSLWCLVKGFYPSDIAVEWESNGQPENNYKTTPPVLDSDGSFFLYSKLTVDKSRWQQGNVFSCSVMHEALHNHYTQKSLSLSPGGSGATNFSLLKQAGDVEENPGPMAIIYLILLFTAVRGIKEEHVIIQAEFYLNPDQSGEFMFDFDGDEIFHVDMAKKETVWRLEEFGRFASFEAQGALANIAVDKANLEIMTKRSNYTPITNVPPEVTVLTNSPVELREPNVLICFIDKFTPPVVNVTWLRNGKPVTTGVSETVFLPREDHLFRKFHYLPFLPSTEDVYDCRVEHWGLDEPLLKHWEFDAPSPLPETTESGGGGGDKTHTCPPCPAPELLGGPSVFLFPPKPKDTLMISRTPEVTCVVVDVSHEDPEVKFNWYVDGVEVHNAKTKPREEQYNSTYRVVSVLTVLHQDWLNGKEYKCKVSNKALPAPIEKTISKAKGQPREPQVCTLPPSRDELTKNQVSLSCAVKGFYPSDIAVEWESNGQPENNYKTTPPVLDSDGSFFLVSKLTVDKSRWQQGNVFSCSVMHEALHNHYTQKSLSLSPGGSGSGSGSLGGIFEAMKMELRDHHHHHHNWSHPQFEKC

SEQ ID NO: 33 - protein, 1055 aa, Artificial Sequence
  source: /note="Description of Artificial Sequence: Synthetic polypeptide"
MAIIYLILLFTAVRGRSAHHPIWARMDAGGGGSLVPRGSGGGGSGDSERHFVHQFKGECYFTNGTQRIRLVTRYIYNREEYLRFDSDVGEYRAVTELGRHSAEYYNKQYLERTRAELDTACRHNYEETEVPTSLRRLEQPNVAISLSRTEALNHHNTLVCSVTDFYPAKIKVRWFRNGQEETVGVSSTQLIRNGDWTFQVLVMLEMTPHQGEVYTCHVEHPSLKSPITVEWRAQSESARSKSGGGGGRIARLEEKVKTLKAQNSELASTANMLREQVAQLKQKVMNHDKTHTCPPCPAPELLGGPSVFLFPPKPKDTLMISRTPEVTCVVVDVSHEDPEVKFNWYVDGVEVHNAKTKPREEQYNSTYRVVSVLTVLHQDWLNGKEYKCKVSNKALPAPIEKTISKAKGQPREPQVYTLPPCRDELTKNQVSLWCLVKGFYPSDIAVEWESNGQPENNYKTTPPVLDSDGSFFLYSKLTVDKSRWQQGNVFSCSVMHEALHNHYTQKSLSLSPGGSGATNFSLLKQAGDVEENPGPMAIIYLILLFTAVRGEDDIEADHVGFYGTTVYQSPGDIGQYTHEFDGDELFYVDLDKKKTVWRLPEFGQLILFEPQGGLQNIAAEKHNLGILTKRSNFTPATNEAPQATVFPKSPVLLGQPNTLICFVDNIFPPVINITWLRNSKSVTDGVYETSFLVNRDHSFHKLSYLTFIPSDDDIYDCKVEHWGLEEPVLKHWEPEIPAPMSELTESGGGGGLTDTLQAETDQLEDEKSALQTEIANLLKEKEKLEFILAAHDKTHTCPPCPAPELLGGPSVFLFPPKPKDTLMISRTPEVTCVVVDVSHEDPEVKFNWYVDGVEVHNAKTKPREEQYNSTYRVVSVLTVLHQDWLNGKEYKCKVSNKALPAPIEKTISKAKGQPREPQVCTLPPSRDELTKNQVSLSCAVKGFYPSDIAVEWESNGQPENNYKTTPPVLDSDGSFFLVSKLTVDKSRWQQGNVFSCSVMHEALHNHYTQKSLSLSPGGSGSGSGSLGGIFEAMKMELRDHHHHHHNWSHPQFEKC

SEQ ID NO: 34 - protein, 975 aa, Artificial Sequence
  source: /note="Description of Artificial Sequence: Synthetic polypeptide"
MAIIYLILLFTAVRGRSAHHPIWARMDAGGGGSLVPRGSGGGGSGDSERHFVHQFKGECYFTNGTQRIRLVTRYIYNREEYLRFDSDVGEYRAVTELGRHSAEYYNKQYLERTRAELDTACRHNYEETEVPTSLRRLEQPNVAISLSRTEALNHHNTLVCSVTDFYPAKIKVRWFRNGQEETVGVSSTQLIRNGDWTFQVLVMLEMTPHQGEVYTCHVEHPSLKSPITVEWRAQSESARSKSGGGGGDKTHTCPPCPAPELLGGPSVFLFPPKPKDTLMISRTPEVTCVVVDVSHEDPEVKFNWYVDGVEVHNAKTKPREEQYNSTYRVVSVLTVLHQDWLNGKEYKCKVSNKALPAPIEKTISKAKGQPREPQVYTLPPCRDELTKNQVSLWCLVKGFYPSDIAVEWESNGQPENNYKTTPPVLDSDGSFFLYSKLTVDKSRWQQGNVFSCSVMHEALHNHYTQKSLSLSPGGSGATNFSLLKQAGDVEENPGPMAIIYLILLFTAVRGEDDIEADHVGFYGTTVYQSPGDIGQYTHEFDGDELFYVDLDKKKTVWRLPEFGQLILFEPQGGLQNIAAEKHNLGILTKRSNFTPATNEAPQATVFPKSPVLLGQPNTLICFVDNIFPPVINITWLRNSKSVTDGVYETSFLVNRDHSFHKLSYLTFIPSDDDIYDCKVEHWGLEEPVLKHWEPEIPAPMSELTESGGGGGDKTHTCPPCPAPELLGGPSVFLFPPKPKDTLMISRTPEVTCVVVDVSHEDPEVKFNWYVDGVEVHNAKTKPREEQYNSTYRVVSVLTVLHQDWLNGKEYKCKVSNKALPAPIEKTISKAKGQPREPQVCTLPPSRDELTKNQVSLSCAVKGFYPSDIAVEWESNGQPENNYKTTPPVLDSDGSFFLVSKLTVDKSRWQQGNVFSCSVMHEALHNHYTQKSLSLSPGGSGSGSGSLGGIFEAMKMELRDHHHHHHNWSHPQFEKC

SEQ ID NO: 35 - protein, 518 aa, Artificial Sequence
  source: /note="Description of Artificial Sequence: Synthetic polypeptide"
MGSLQPLATLYLLGMLVASSLGQHLQKDYRAYYTFGGGGGSGGGSGGSGDTRPRFLEYSTSECHFFNGTERVRYLDRYFHNQEENVRFDSDVGEFRAVTELGRPDAEYWNSQKDLLEQKRGRVDNYCRHNYGVVESFTVQRRVHPKVTVYPSKTQPLQHHNLLVCSVSGFYPGSIEVRWFRNGQEEKTGVVSTGLIHNGDWTFQTLVMLETVPRSGEVYTCQVEHPSVTSPLTVEWRARSESAQSKSGGGGGRIARLEEKVKTLKAQNSELASTANMLREQVAQLKQKVMNHDKTHTCPPCPAPELLGGPSVFLFPPKPKDTLMISRTPEVTCVVVDVSHEDPEVKFNWYVDGVEVHNAKTKPREEQYNSTYRVVSVLTVLHQDWLNGKEYKCKVSNKALPAPIEKTISKAKGQPREPQVCTLPPSRDELTKNQVSLSCAVKGFYPSDIAVEWESNGQPENNYKTTPPVLDSDGSFFLVSKLTVDKSRWQQGNVFSCSVMHEALHNHYTQKSLSLSPG

SEQ ID NO: 36 - protein, 518 aa, Artificial Sequence
  source: /note="Description of Artificial Sequence: Synthetic polypeptide"
MGSLQPLATLYLLGMLVASSLGQHLQKDYRAYYTFGGGGGSGGGSGGSGDTRPRFLEYSTSECHFFNGTERVRYLDRYFHNQEENVRFDSDVGEFRAVTELGRPDAEYWNSQKDLLEQKRGRVDNYCRHNYGVVESFTVQRRVHPKVTVYPSKTQPLQHHNLLVCSVSGFYPGSIEVRWFRNGQEEKTGVVSTGLIHNGDWTFQTLVMLETVPRSGEVYTCQVEHPSVTSPLTVEWRARSESAQSKSGGGGGRIARLEEKVKTLKAQNSELASTANMLREQVAQLKQKVMNHDKTHTCPPCPAPELLGGPSVFLFPPKPKDTLMISRTPEVTCVVVDVSHEDPEVKFNWYVDGVEVHNAKTKPREEQYNSTYRVVSVLTVLHQDWLNGKEYKCKVSNKALPAPIEKTISKAKGQPREPQVYTLPPCRDELTKNQVSLWCLVKGFYPSDIAVEWESNGQPENNYKTTPPVLDSDGSFFLYSKLTVDKSRWQQGNVFSCSVMHEALHNHYTQKSLSLSPG

SEQ ID NO: 37 - protein, 478 aa, Artificial Sequence
  source: /note="Description of Artificial Sequence: Synthetic polypeptide"
MAIIYLILLFTAVRGIKEEHVIIQAEFYLNPDQSGEFMFDFDGDEIFHVDMAKKETVWRLEEFGRFASFEAQGALANIAVDKANLEIMTKRSNYTPITNVPPEVTVLTNSPVELREPNVLICFIDKFTPPVVNVTWLRNGKPVTTGVSETVFLPREDHLFRKFHYLPFLPSTEDVYDCRVEHWGLDEPLLKHWEFDAPSPLPETTESGGGGGLTDTLQAETDQLEDEKSALQTEIANLLKEKEKLEFILAAHDKTHTCPPCPAPELLGGPSVFLFPPKPKDTLMISRTPEVTCVVVDVSHEDPEVKFNWYVDGVEVHNAKTKPREEQYNSTYRVVSVLTVLHQDWLNGKEYKCKVSNKALPAPIEKTISKAKGQPREPQVYTLPPCRDELTKNQVSLWCLVKGFYPSDIAVEWESNGQPENNYKTTPPVLDSDGSFFLYSKLTVDKSRWQQGNVFSCSVMHEALHNHYTQKSLSLSPG

SEQ ID NO: 38 - protein, 478 aa, Artificial Sequence
  source: /note="Description of Artificial Sequence: Synthetic polypeptide"
MAIIYLILLFTAVRGIKEEHVIIQAEFYLNPDQSGEFMFDFDGDEIFHVDMAKKETVWRLEEFGRFASFEAQGALANIAVDKANLEIMTKRSNYTPITNVPPEVTVLTNSPVELREPNVLICFIDKFTPPVVNVTWLRNGKPVTTGVSETVFLPREDHLFRKFHYLPFLPSTEDVYDCRVEHWGLDEPLLKHWEFDAPSPLPETTESGGGGGLTDTLQAETDQLEDEKSALQTEIANLLKEKEKLEFILAAHDKTHTCPPCPAPELLGGPSVFLFPPKPKDTLMISRTPEVTCVVVDVSHEDPEVKFNWYVDGVEVHNAKTKPREEQYNSTYRVVSVLTVLHQDWLNGKEYKCKVSNKALPAPIEKTISKAKGQPREPQVCTLPPSRDELTKNQVSLSCAVKGFYPSDIAVEWESNGQPENNYKTTPPVLDSDGSFFLVSKLTVDKSRWQQGNVFSCSVMHEALHNHYTQKSLSLSPG

SEQ ID NO: 39 - protein, 478 aa, Artificial Sequence
  source: /note="Description of Artificial Sequence: Synthetic polypeptide"
MGSLQPLATLYLLGMLVASSLGQHLQKDYRAYYTFGGGGGSGGGSGGSGDTRPRFLEYSTSECHFFNGTERVRYLDRYFHNQEENVRFDSDVGEFRAVTELGRPDAEYWNSQKDLLEQKRGRVDNYCRHNYGVVESFTVQRRVHPKVTVYPSKTQPLQHHNLLVCSVSGFYPGSIEVRWFRNGQEEKTGVVSTGLIHNGDWTFQTLVMLETVPRSGEVYTCQVEHPSVTSPLTVEWRARSESAQSKSGGGGGDKTHTCPPCPAPELLGGPSVFLFPPKPKDTLMISRTPEVTCVVVDVSHEDPEVKFNWYVDGVEVHNAKTKPREEQYNSTYRVVSVLTVLHQDWLNGKEYKCKVSNKALPAPIEKTISKAKGQPREPQVCTLPPSRDELTKNQVSLSCAVKGFYPSDIAVEWESNGQPENNYKTTPPVLDSDGSFFLVSKLTVDKSRWQQGNVFSCSVMHEALHNHYTQKSLSLSPG

SEQ ID NO: 40 - protein, 478 aa, Artificial Sequence
  source: /note="Description of Artificial Sequence: Synthetic polypeptide"
MGSLQPLATLYLLGMLVASSLGQHLQKDYRAYYTFGGGGGSGGGSGGSGDTRPRFLEYSTSECHFFNGTERVRYLDRYFHNQEENVRFDSDVGEFRAVTELGRPDAEYWNSQKDLLEQKRGRVDNYCRHNYGVVESFTVQRRVHPKVTVYPSKTQPLQHHNLLVCSVSGFYPGSIEVRWFRNGQEEKTGVVSTGLIHNGDWTFQTLVMLETVPRSGEVYTCQVEHPSVTSPLTVEWRARSESAQSKSGGGGGDKTHTCPPCPAPELLGGPSVFLFPPKPKDTLMISRTPEVTCVVVDVSHEDPEVKFNWYVDGVEVHNAKTKPREEQYNSTYRVVSVLTVLHQDWLNGKEYKCKVSNKALPAPIEKTISKAKGQPREPQVYTLPPCRDELTKNQVSLWCLVKGFYPSDIAVEWESNGQPENNYKTTPPVLDSDGSFFLYSKLTVDKSRWQQGNVFSCSVMHEALHNHYTQKSLSLSPG

SEQ ID NO: 41 - protein, 438 aa, Artificial Sequence
  source: /note="Description of Artificial Sequence: Synthetic polypeptide"
MAIIYLILLFTAVRGIKEEHVIIQAEFYLNPDQSGEFMFDFDGDEIFHVDMAKKETVWRLEEFGRFASFEAQGALANIAVDKANLEIMTKRSNYTPITNVPPEVTVLTNSPVELREPNVLICFIDKFTPPVVNVTWLRNGKPVTTGVSETVFLPREDHLFRKFHYLPFLPSTEDVYDCRVEHWGLDEPLLKHWEFDAPSPLPETTESGGGGGDKTHTCPPCPAPELLGGPSVFLFPPKPKDTLMISRTPEVTCVVVDVSHEDPEVKFNWYVDGVEVHNAKTKPREEQYNSTYRVVSVLTVLHQDWLNGKEYKCKVSNKALPAPIEKTISKAKGQPREPQVYTLPPCRDELTKNQVSLWCLVKGFYPSDIAVEWESNGQPENNYKTTPPVLDSDGSFFLYSKLTVDKSRWQQGNVFSCSVMHEALHNHYTQKSLSLSPG

SEQ ID NO: 42 - protein, 438 aa, Artificial Sequence
  source: /note="Description of Artificial Sequence: Synthetic polypeptide"
MAIIYLILLFTAVRGIKEEHVIIQAEFYLNPDQSGEFMFDFDGDEIFHVDMAKKETVWRLEEFGRFASFEAQGALANIAVDKANLEIMTKRSNYTPITNVPPEVTVLTNSPVELREPNVLICFIDKFTPPVVNVTWLRNGKPVTTGVSETVFLPREDHLFRKFHYLPFLPSTEDVYDCRVEHWGLDEPLLKHWEFDAPSPLPETTESGGGGGDKTHTCPPCPAPELLGGPSVFLFPPKPKDTLMISRTPEVTCVVVDVSHEDPEVKFNWYVDGVEVHNAKTKPREEQYNSTYRVVSVLTVLHQDWLNGKEYKCKVSNKALPAPIEKTISKAKGQPREPQVCTLPPSRDELTKNQVSLSCAVKGFYPSDIAVEWESNGQPENNYKTTPPVLDSDGSFFLVSKLTVDKSRWQQGNVFSCSVMHEALHNHYTQKSLSLSPG

SEQ ID NO: 43 - protein, 513 aa, Artificial Sequence
  source: /note="Description of Artificial Sequence: Synthetic polypeptide"
MAIIYLILLFTAVRGRSAHHPIWARMDAGGGGSLVPRGSGGGGSGDSERHFVHQFKGECYFTNGTQRIRLVTRYIYNREEYLRFDSDVGEYRAVTELGRHSAEYYNKQYLERTRAELDTACRHNYEETEVPTSLRRLEQPNVAISLSRTEALNHHNTLVCSVTDFYPAKIKVRWFRNGQEETVGVSSTQLIRNGDWTFQVLVMLEMTPHQGEVYTCHVEHPSLKSPITVEWRAQSESARSKSGGGGGRIARLEEKVKTLKAQNSELASTANMLREQVAQLKQKVMNHDKTHTCPPCPAPELLGGPSVFLFPPKPKDTLMISRTPEVTCVVVDVSHEDPEVKFNWYVDGVEVHNAKTKPREEQYNSTYRVVSVLTVLHQDWLNGKEYKCKVSNKALPAPIEKTISKAKGQPREPQVCTLPPSRDELTKNQVSLSCAVKGFYPSDIAVEWESNGQPENNYKTTPPVLDSDGSFFLVSKLTVDKSRWQQGNVFSCSVMHEALHNHYTQKSLSLSPG

SEQ ID NO: 44 - protein, 513 aa, Artificial Sequence
  source: /note="Description of Artificial Sequence: Synthetic polypeptide"
MAIIYLILLFTAVRGRSAHHPIWARMDAGGGGSLVPRGSGGGGSGDSERHFVHQFKGECYFTNGTQRIRLVTRYIYNREEYLRFDSDVGEYRAVTELGRHSAEYYNKQYLERTRAELDTACRHNYEETEVPTSLRRLEQPNVAISLSRTEALNHHNTLVCSVTDFYPAKIKVRWFRNGQEETVGVSSTQLIRNGDWTFQVLVMLEMTPHQGEVYTCHVEHPSLKSPITVEWRAQSESARSKSGGGGGRIARLEEKVKTLKAQNSELASTANMLREQVAQLKQKVMNHDKTHTCPPCPAPELLGGPSVFLFPPKPKDTLMISRTPEVTCVVVDVSHEDPEVKFNWYVDGVEVHNAKTKPREEQYNSTYRVVSVLTVLHQDWLNGKEYKCKVSNKALPAPIEKTISKAKGQPREPQVYTLPPCRDELTKNQVSLWCLVKGFYPSDIAVEWESNGQPENNYKTTPPVLDSDGSFFLYSKLTVDKSRWQQGNVFSCSVMHEALHNHYTQKSLSLSPG

SEQ ID NO: 45 - protein, 482 aa, Artificial Sequence
  source: /note="Description of Artificial Sequence: Synthetic polypeptide"
MAIIYLILLFTAVRGEDDIEADHVGFYGTTVYQSPGDIGQYTHEFDGDELFYVDLDKKKTVWRLPEFGQLILFEPQGGLQNIAAEKHNLGILTKRSNFTPATNEAPQATVFPKSPVLLGQPNTLICFVDNIFPPVINITWLRNSKSVTDGVYETSFLVNRDHSFHKLSYLTFIPSDDDIYDCKVEHWGLEEPVLKHWEPEIPAPMSELTESGGGGGLTDTLQAETDQLEDEKSALQTEIANLLKEKEKLEFILAAHDKTHTCPPCPAPELLGGPSVFLFPPKPKDTLMISRTPEVTCVVVDVSHEDPEVKFNWYVDGVEVHNAKTKPREEQYNSTYRVVSVLTVLHQDWLNGKEYKCKVSNKALPAPIEKTISKAKGQPREPQVYTLPPCRDELTKNQVSLWCLVKGFYPSDIAVEWESNGQPENNYKTTPPVLDSDGSFFLYSKLTVDKSRWQQGNVFSCSVMHEALHNHYTQKSLSLSPG

SEQ ID NO: 46 - protein, 482 aa, Artificial Sequence
  source: /note="Description of Artificial Sequence: Synthetic polypeptide"
MAIIYLILLFTAVRGEDDIEADHVGFYGTTVYQSPGDIGQYTHEFDGDELFYVDLDKKKTVWRLPEFGQLILFEPQGGLQNIAAEKHNLGILTKRSNFTPATNEAPQATVFPKSPVLLGQPNTLICFVDNIFPPVINITWLRNSKSVTDGVYETSFLVNRDHSFHKLSYLTFIPSDDDIYDCKVEHWGLEEPVLKHWEPEIPAPMSELTESGGGGGLTDTLQAETDQLEDEKSALQTEIANLLKEKEKLEFILAAHDKTHTCPPCPAPELLGGPSVFLFPPKPKDTLMISRTPEVTCVVVDVSHEDPEVKFNWYVDGVEVHNAKTKPREEQYNSTYRVVSVLTVLHQDWLNGKEYKCKVSNKALPAPIEKTISKAKGQPREPQVCTLPPSRDELTKNQVSLSCAVKGFYPSDIAVEWESNGQPENNYKTTPPVLDSDGSFFLVSKLTVDKSRWQQGNVFSCSVMHEALHNHYTQKSLSLSPG

SEQ ID NO: 47 - protein, 473 aa, Artificial Sequence
  source: /note="Description of Artificial Sequence: Synthetic polypeptide"
MAIIYLILLFTAVRGRSAHHPIWARMDAGGGGSLVPRGSGGGGSGDSERHFVHQFKGECYFTNGTQRIRLVTRYIYNREEYLRFDSDVGEYRAVTELGRHSAEYYNKQYLERTRAELDTACRHNYEETEVPTSLRRLEQPNVAISLSRTEALNHHNTLVCSVTDFYPAKIKVRWFRNGQEETVGVSSTQLIRNGDWTFQVLVMLEMTPHQGEVYTCHVEHPSLKSPITVEWRAQSESARSKSGGGGGDKTHTCPPCPAPELLGGPSVFLFPPKPKDTLMISRTPEVTCVVVDVSHEDPEVKFNWYVDGVEVHNAKTKPREEQYNSTYRVVSVLTVLHQDWLNGKEYKCKVSNKALPAPIEKTISKAKGQPREPQVCTLPPSRDELTKNQVSLSCAVKGFYPSDIAVEWESNGQPENNYKTTPPVLDSDGSFFLVSKLTVDKSRWQQGNVFSCSVMHEALHNHYTQKSLSLSPG

SEQ ID NO: 48 - protein, 473 aa, Artificial Sequence
  source: /note="Description of Artificial Sequence: Synthetic polypeptide"
MAIIYLILLFTAVRGRSAHHPIWARMDAGGGGSLVPRGSGGGGSGDSERHFVHQFKGECYFTNGTQRIRLVTRYIYNREEYLRFDSDVGEYRAVTELGRHSAEYYNKQYLERTRAELDTACRHNYEETEVPTSLRRLEQPNVAISLSRTEALNHHNTLVCSVTDFYPAKIKVRWFRNGQEETVGVSSTQLIRNGDWTFQVLVMLEMTPHQGEVYTCHVEHPSLKSPITVEWRAQSESARSKSGGGGGDKTHTCPPCPAPELLGGPSVFLFPPKPKDTLMISRTPEVTCVVVDVSHEDPEVKFNWYVDGVEVHNAKTKPREEQYNSTYRVVSVLTVLHQDWLNGKEYKCKVSNKALPAPIEKTISKAKGQPREPQVYTLPPCRDELTKNQVSLWCLVKGFYPSDIAVEWESNGQPENNYKTTPPVLDSDGSFFLYSKLTVDKSRWQQGNVFSCSVMHEALHNHYTQKSLSLSPG

SEQ ID NO: 49 - protein, 442 aa, Artificial Sequence
  source: /note="Description of Artificial Sequence: Synthetic polypeptide"
MAIIYLILLFTAVRGEDDIEADHVGFYGTTVYQSPGDIGQYTHEFDGDELFYVDLDKKKTVWRLPEFGQLILFEPQGGLQNIAAEKHNLGILTKRSNFTPATNEAPQATVFPKSPVLLGQPNTLICFVDNIFPPVINITWLRNSKSVTDGVYETSFLVNRDHSFHKLSYLTFIPSDDDIYDCKVEHWGLEEPVLKHWEPEIPAPMSELTESGGGGGDKTHTCPPCPAPELLGGPSVFLFPPKPKDTLMISRTPEVTCVVVDVSHEDPEVKFNWYVDGVEVHNAKTKPREEQYNSTYRVVSVLTVLHQDWLNGKEYKCKVSNKALPAPIEKTISKAKGQPREPQVYTLPPCRDELTKNQVSLWCLVKGFYPSDIAVEWESNGQPENNYKTTPPVLDSDGSFFLYSKLTVDKSRWQQGNVFSCSVMHEALHNHYTQKSLSLSPG

SEQ ID NO: 50 - protein, 442 aa, Artificial Sequence
  source: /note="Description of Artificial Sequence: Synthetic polypeptide"
MAIIYLILLFTAVRGEDDIEADHVGFYGTTVYQSPGDIGQYTHEFDGDELFYVDLDKKKTVWRLPEFGQLILFEPQGGLQNIAAEKHNLGILTKRSNFTPATNEAPQATVFPKSPVLLGQPNTLICFVDNIFPPVINITWLRNSKSVTDGVYETSFLVNRDHSFHKLSYLTFIPSDDDIYDCKVEHWGLEEPVLKHWEPEIPAPMSELTESGGGGGDKTHTCPPCPAPELLGGPSVFLFPPKPKDTLMISRTPEVTCVVVDVSHEDPEVKFNWYVDGVEVHNAKTKPREEQYNSTYRVVSVLTVLHQDWLNGKEYKCKVSNKALPAPIEKTISKAKGQPREPQVCTLPPSRDELTKNQVSLSCAVKGFYPSDIAVEWESNGQPENNYKTTPPVLDSDGSFFLVSKLTVDKSRWQQGNVFSCSVMHEALHNHYTQKSLSLSPG

SEQ ID NO: 51 - protein, 226 aa, Artificial Sequence
  source: /note="Description of Artificial Sequence: Synthetic polypeptide"
DKTHTCPPCPAPELLGGPSVFLFPPKPKDTLMISRTPEVTCVVVDVSHEDPEVKFNWYVDGVEVHNAKTKPREEQYNSTYRVVSVLTVLHQDWLNGKEYKCKVSNKALPAPIEKTISKAKGQPREPQVCTLPPSRDELTKNQVSLSCAVKGFYPSDIAVEWESNGQPENNYKTTPPVLDSDGSFFLVSKLTVDKSRWQQGNVFSCSVMHEALHNHYTQKSLSLSPG

SEQ ID NO: 52 - protein, 106 aa, Homo sapiens
GQPREPQVCTLPPSRDELTKNQVSLSCAVKGFYPSDIAVEWESNGQPENNYKTTPPVLDSDGSFFLVSKLTVDKSRWQQGNVFSCSVMHEALHNHYTQKSLSLSPG

SEQ ID NO: 53 - protein, 226 aa, Artificial Sequence
  source: /note="Description of Artificial Sequence: Synthetic polypeptide"
DKTHTCPPCPAPELLGGPSVFLFPPKPKDTLMISRTPEVTCVVVDVSHEDPEVKFNWYVDGVEVHNAKTKPREEQYNSTYRVVSVLTVLHQDWLNGKEYKCKVSNKALPAPIEKTISKAKGQPREPQVYTLPPCRDELTKNQVSLWCLVKGFYPSDIAVEWESNGQPENNYKTTPPVLDSDGSFFLYSKLTVDKSRWQQGNVFSCSVMHEALHNHYTQKSLSLSPG

SEQ ID NO: 54 - protein, 106 aa, Homo sapiens
GQPREPQVYTLPPCRDELTKNQVSLWCLVKGFYPSDIAVEWESNGQPENNYKTTPPVLDSDGSFFLYSKLTVDKSRWQQGNVFSCSVMHEALHNHYTQKSLSLSPG

SEQ ID NO: 55 - protein, 113 aa, Homo sapiens
PCPAPELLGGPSVFLFPPKPKDTLMISRTPEVTCVVVDVSHEDPEVKFNWYVDGVEVHNAKTKPREEQYNSTYRVVSVLTVLHQDWLNGKEYKCKVSNKALPAPIEKTISKAK

SEQ ID NO: 56 - protein, 224 aa, Artificial Sequence
  source: /note="Description of Artificial Sequence: Synthetic polypeptide"
QHLQKDYRAYYTFGGGGGSGGGSGGSGDTRPRFLEYSTSECHFFNGTERVRYLDRYFHNQEENVRFDSDVGEFRAVTELGRPDAEYWNSQKDLLEQKRGRVDNYCRHNYGVVESFTVQRRVHPKVTVYPSKTQPLQHHNLLVCSVSGFYPGSIEVRWFRNGQEEKTGVVSTGLIHNGDWTFQTLVMLETVPRSGEVYTCQVEHPSVTSPLTVEWRARSESAQSK

SEQ ID NO: 57 - protein, 191 aa, Homo sapiens
IKEEHVIIQAEFYLNPDQSGEFMFDFDGDEIFHVDMAKKETVWRLEEFGRFASFEAQGALANIAVDKANLEIMTKRSNYTPITNVPPEVTVLTNSPVELREPNVLICFIDKFTPPVVNVTWLRNGKPVTTGVSETVFLPREDHLFRKFHYLPFLPSTEDVYDCRVEHWGLDEPLLKHWEFDAPSPLPETTE

SEQ ID NO: 58 - protein, 198 aa, Mus musculus
GDSERHFVHQFKGECYFTNGTQRIRLVTRYIYNREEYLRFDSDVGEYRAVTELGRHSAEYYNKQYLERTRAELDTACRHNYEETEVPTSLRRLEQPNVAISLSRTEALNHHNTLVCSVTDFYPAKIKVRWFRNGQEETVGVSSTQLIRNGDWTFQVLVMLEMTPHQGEVYTCHVEHPSLKSPITVEWRAQSESARSKS

SEQ ID NO: 59 - protein, 196 aa, Mus musculus
EDDIEADHVGFYGTTVYQSPGDIGQYTHEFDGDELFYVDLDKKKTVWRLPEFGQLILFEPQGGLQNIAAEKHNLGILTKRSNFTPATNEAPQATVFPKSPVLLGQPNTLICFVDNIFPPVINITWLRNSKSVTDGVYETSFLVNRDHSFHKLSYLTFIPSDDDIYDCKVEHWGLEEPVLKHWEPEIPAPMSELTES

SEQ ID NO: 60 - protein, 476 aa, Artificial Sequence
  source: /note="Description of Artificial Sequence: Synthetic polypeptide"
MAIIYLILLFTAVRGIKEEHVIIQAEFYLNPDQSGEFMFDFDGDEIFHVDMAKKETVWRLEEFGRFASFEAQGALANIAVDKANLECMTKRSNYTPITNVPPEVTVLTNSPVELREPNVLICFIDKFTPPVVNVTWLRNGKPVTTGVSETVFLPREDHLFRKFHYLPFLPSTEDVYDCRVEHWGLDEPLLKHWEFDAPSPLPETTESGGGGGDKTHTCPPCPAPELLGGPSVFLFPPKPKDTLMISRTPEVTCVVVDVSHEDPEVKFNWYVDGVEVHNAKTKPREEQYNSTYRVVSVLTVLHQDWLNGKEYKCKVSNKALPAPIEKTISKAKGQPREPQVYTLPPCRDELTKNQVSLWCLVKGFYPSDIAVEWESNGQPENNYKTTPPVLDSDGSFFLYSKLTVDKSRWQQGNVFSCSVMHEALHNHYTQKSLSLSPGGSGSGSGSLGGIFEAMKMELRDHHHHHHNWSHPQFEKC

SEQ ID NO: 61 - protein, 478 aa, Artificial Sequence
  source: /note="Description of Artificial Sequence: Synthetic polypeptide"
MGSLQPLATLYLLGMLVASSLGQHLQKDYRAYYTCGGGGGSGGGSGGSGDTRPRFLEYSTSECHFFNGTERVRYLDRYFHNQEENVRFDSDVGEFRAVTELGRPDAEYWNSQKDLLEQKRGRVDNYCRHNYGVVESFTVQRRVHPKVTVYPSKTQPLQHHNLLVCSVSGFYPGSIEVRWFRNGQEEKTGVVSTGLIHNGDWTFQTLVMLETVPRSGEVYTCQVEHPSVTSPLTVEWRARSESAQSKSGGGGGDKTHTCPPCPAPELLGGPSVFLFPPKPKDTLMISRTPEVTCVVVDVSHEDPEVKFNWYVDGVEVHNAKTKPREEQYNSTYRVVSVLTVLHQDWLNGKEYKCKVSNKALPAPIEKTISKAKGQPREPQVCTLPPSRDELTKNQVSLSCAVKGFYPSDIAVEWESNGQPENNYKTTPPVLDSDGSFFLVSKLTVDKSRWQQGNVFSCSVMHEALHNHYTQKSLSLSPG

SEQ ID NO: 62 - protein, 443 aa, Artificial Sequence
  source: /note="Description of Artificial Sequence: Synthetic polypeptide"
MMSFVSLLLVGILFHATQAIKEEHVIIQAEFYLNPDQSGEFMFDFDGDEIFHVDMAKKETVWRLEEFGRFASFEAQGALANIAVDKANLEMTKRSNYTPITNVPPEVTVLTNSVELREPNVLICFIDKFTPVVNVTWLRNGKPVTTGVSETVFLPREDHLFRKFHYLPFLPSTEDVYDCRVEHWGLDEPLLKHWEFDAPSPLPETTESGGGGGDKTHTCPCPAPEAAGGPSVFLFPPKPKDTLMISRTPEVTCVVVDVSHEDPEVKFNWYVDGVEVHNAKTKPREEQYNSTYRVVSVLTVLHQDWLNGKEYKCKVSNKALPAPIEKTISKAKGQPREPQVYTLPPCRDELTKNQVSLWCLVKGFYPSDIAVEWESNGQPENNYKTTPPVLDSDGSFFLYSKLTVDKSRWQQGNVFSCSVMHEALHNHYTQKSLSLSPGGSGSC

SEQ ID NO: 63 - protein, 478 aa, Artificial Sequence
  source: /note="Description of Artificial Sequence: Synthetic polypeptide"
MGSLQPLATLYLLGMLVASSLGQHLQKDYRAYYTCGGGGGSGGGSGGSGDTRPRFLEYSTSECHFFNGTERVRYLDRYFHNQEENVRFDSDVGEFRAVTELGRPDAEYWNSQKDLLEQKRGRVDNYCRHNYGVVESFTVQRRVHPKVTVYPSKTQPLQHHNLLVCSVSGFYPGSIEVRWFRNGQEEKTGVVSTGLIHNGDWTFQTLVMLETVPRSGEVYTCQVEHPSVTSPLTVEWRARSESAQSKSGGGGGDKTHTCPPCPAPEAAGGPSVFLFPPKPKDTLMISRTPEVTCVVVDVSHEDPEVKFNWYVDGVEVHNAKTKPREEQYNSTYRVVSVLTVLHQDWLNGKEYKCKVSNKALPAPIEKTISKAKGQPREPQVCTLPPSRDELTKNQVSLSCAVKGFYPSDIAVEWESNGQPENNYKTTPPVLDSDGSFFLVSKLTVDKSRWQQGNVFSCSVMHEALHNHYTQKSLSLSPG

SEQ ID NO: 64 - DNA, 1344 bp, Artificial Sequence
  source: /note="Description of Artificial Sequence: Synthetic polynucleotide"
atgatgagcttcgtgagcctgctgctggtgggcatcctgttccacgccacccaggccatcaaagaagaacatgtgatcatccaggccgagttctatctgaatcctgaccaatcaggcgagtttatgtttgactttgatggtgatgagattttccatgtggatatggcaaagaaggagacggtctggcggcttgaagaatttggacgatttgccagctttgaggctcaaggtgcattggccaacatagctgtggacaaagccaacctggaatgcatgacaaagcgctccaactatactccgatcaccaatgtacctccagaggtaactgtgctcacaaacagccctgtggaactgagagagcccaacgtcctcatctgtttcatagacaagttcaccccaccagtggtcaatgtcacgtggcttcgaaatggaaaacctgtcaccacaggagtgtcagagacagtcttcctgcccagggaagaccaccttttccgcaagttccactatctccccttcctgccctcaactgaggacgtttacgactgcagggtggagcactggggcttggatgagcctcttctcaagcactgggagtttgatgctccaagccctctcccagagactacagagtccggaggcggaggcggagacaaaactcacacatgcccaccgtgcccagcacctgaagccgcggggggaccgtcagtcttcctcttccccccaaaacccaaggacaccctcatgatctcccggacccctgaggtcacatgcgtggtggtggacgtgagccacgaagaccctgaggtcaagttcaactggtacgtggacggcgtggaggtgcataatgccaagacaaagccgcgggaggagcagtacaacagcacgtaccgtgtggtcagcgtcctcaccgtcctgcaccaggactggctgaatggcaaggagtacaagtgcaaggtctccaacaaagccctcccagcccccatcgagaaaaccatctccaaagccaaagggcagccccgagaaccacaggtgtacaccctgcccccatgccgggatgagctgaccaagaaccaggtcagcctgtggtgcctggtcaaaggcttctatcccagcgacatcgccgtggagtgggagagcaatgggcagccggagaacaactacaagaccacgcctcccgtgctggactccgacggctccttcttcctctacagcaagctcaccgtggacaagagtaggtggcagcaggggaacgtcttctcatgctccgtgatgcatgaggctctgcacaaccactacacacagaagagcctctccctgtctccgggcggtagtggtagttgttga

SEQ ID NO: 65 - DNA, 1437 bp, Artificial Sequence
  source: /note="Description of Artificial Sequence: Synthetic polynucleotide"
atgggttctctgcaaccgctggccaccttgtacctgctgggtatgctggtcgctagcagcctcggacagcacctgcagaaggactacagagcctactacacctgtggaggtggaggcggctcaggaggtggaagcggcggctctggggacacccgaccacgtttcttggagtactctacgtctgagtgtcatttcttcaatgggacggagcgggtgcggtacctggacagatacttccataaccaggaggagaacgtgcgcttcgacagcgacgtgggggagttccgggcggtgacggagctggggcggcctgatgccgagtactggaacagccagaaggacctcctggagcagaagcggggccgggtggacaactactgcagacacaactacggggttgtggagagcttcacagtgcagcggcgagtccatcctaaggtgactgtgtatccttcaaagacccagcccctgcagcaccataacctcctggtctgttctgtgagtggtttctatccaggcagcattgaagtcaggtggttccggaatggccaggaagagaagactggggtggtgtccacaggcctgatccacaatggagactggaccttccagaccctggtgatgctggaaacagttcctcggagtggagaggtttacacctgccaagtggagcacccaagcgtgacaagccctctcacagtggaatggagagcacggtctgaatctgcacagagcaagtccggaggcggaggcggagacaaaactcacacatgcccaccgtgcccagcacctgaagccgcggggggaccgtcagtcttcctcttccccccaaaacccaaggacaccctcatgatctcccggacccctgaggtcacatgcgtggtggtggacgtgagccacgaagaccctgaggtcaagttcaactggtacgtggacggcgtggaggtgcataatgccaagacaaagccgcgggaggagcagtacaacagcacgtaccgtgtggtcagcgtcctcaccgtcctgcaccaggactggctgaatggcaaggagtacaagtgcaaagtctccaacaaagccctcccagcccccatcgagaaaaccatctccaaagccaaagggcagccccgagaaccacaggtgtgcaccctgcccccatcccgggatgagctgaccaagaaccaggtcagcctgagctgcgcggtcaaaggcttctatcccagcgacatcgccgtggagtgggagagcaatgggcagccggagaacaactacaagaccacgcctcccgtgctggactccgacggctccttcttcctcgtcagcaagctcaccgtggacaagagcaggtggcagcaggggaacgtcttctcatgctccgtgatgcatgaggctctgcacaaccactacacacagaagagcctctccctgtctcccggctga